European Patent Application EP 4 603 513 A1, published August 20, 2025. Title: USE OF ANTIBODY MUTATION METHOD FOR THERAPEUTIC ANTIBODY DRUG. Applicant: SHENZHEN BAISHITONG TECHNOLOGY DEVELOPMENT COMPANY LIMITED. Application US. The sequence listing filed with the application follows.

SEQUENCE LISTING (147 sequences)

SEQ ID NO: 1 - protein, 133 aa, Artificial sequence [sequence omitted]

SEQ ID NO: 2 - protein, 133 aa, Artificial sequence
APTSSSTKKTQLQLEHLLLDLQMILNGINNYKNPKLTRMLTFKFYMPKKATELKHLQCLEEELKPLEEVLNLAQSKNFHLRPRDLISNINVIVLELKGSETTFMSEYADETATIVEFLNRWITFCQSIISTLT

SEQ ID NO: 3 - protein, 133 aa, Artificial sequence
APTSSSTKKTQLQLEHLLLDLQMILNGINNYKNPKLTRMLTAKFYMPKKATELKHLQCLEEELKPLEEVLNLAQSKNFHLRPRDLISNINVIVLELKGSETTFMSEYADETATIVEFLNRWITFAQSIISTLT

SEQ ID NO: 4 - protein, 133 aa, Artificial sequence
APTSSSTKKTQLQLEHLLLDLQMILNGINNYKNPKLTRMLTFKFYMPKKATELKHLQCLEEELKPLEEVLNLAQSKNFHFDPRDVVSNINVFVLELKGSETTFMSEYADETATIVEFLNRWITFAQSIISTLT

SEQ ID NO: 5 - protein, 197 aa, Artificial sequence
RNLPVATPDPGMFPCLHHSQNLLRAVSNMLQKARQTLEFYPCTSEEIDHEDITKDKTSTVEACLPLELTKNESCLNSRETSFITNGSCLASRKTSFMMALCLSSIYEDLKMYQVEFKTMNAKLLMDPKRQIFLDQNMLAVIDELMQALNFNSETVPQKSSLEEPDFYKTKIKLCILLHAFRIRAVTIDRVMSYLNAS

SEQ ID NO: 6 - protein, 193 aa, Artificial sequence
RVIPVSGPARCLSQSRNLLKTTDDMVKTAREKLKHYSCTAEDIDHEDITRDQTSTLKTCLPLELHKNESCLATRETSSTTRGSCLPPQKTSLMMTLCLGSIYEDLKMYQTEFQAINAALQNHNHQQIILDKGMLVAIDELMQSLNHNGETLRQKPPVGEADPYRVKMKLCILLHAFSTRVVTINRVMGYLSSA

SEQ ID NO: 7 - protein, 306 aa, Artificial sequence
IWELKKDVYVVELDWYPDAPGEMVVLTCDTPEEDGITWTLDQSSEVLGSGKTLTIQVKEFGDAGQYTCHKGGEVLSHSLLLLHKKEDGIWSTDILKDQKEPKNKTFLRCEAKNYSGRFTCWWLTTISTDLTFSVKSSRGSSDPQGVTCGAATLSAERVRGDNKEYEYSVECQEDSACPAAEESLPIEVMVDAVHKLKYENYTSSFFIRDIIKPDPPKNLQLKPLKNSRQVEVSWEYPDTWSTPHSYFSLTFCVQVQGKSKREKKDRVFTDKTSATVICRKNASISVRAQDRYYSSSWSEWASVPCS

SEQ ID NO: 8 - protein, 313 aa, Artificial sequence
MWELEKDVYVVEVDWTPDAPGETVNLTCDTPEEDDITWTSDQRHGVIGSGKTLTITVKEFLDAGQYTCHKGGETLSHSHLLLHKKENGIWSTEILKNFKNKTFLKCEAPNYSGRFTCSWLVQRNMDLKFNIKSSSSSPDSRAVTCGMASLSAEKVTLDQRDYEKYSVSCQEDVTCPTAEETLPIELALEARQQNKYENYSTSFFIRDIIKPDPPKNLQMKPLKNSQVEVSWEYPDSWSTPHSYFSLKFFVRIQRKKEKMKETEEGCNQKGAFLVEKTSTEVQCKGGNVCVQAQDRYYNSSCSKWACVPCRVRS

SEQ ID NO: 9 - protein, 522 aa, Artificial sequence
IWELKKDVYVVELDWYPDAPGEMVVLTCDTPEEDGITWTLDQSSEVLGSGKTLTIQVKEFGDAGQYTCHKGGEVLSHSLLLLHKKEDGIWSTDILKDQKEPKNKTFLRCEAKNYSGRFTCWWLTTISTDLTFSVKSSRGSSDPQGVTCGAATLSAERVRGDNKEYEYSVECQEDSACPAAEESLPIEVMVDAVHKLKYENYTSSFFIRDIIKPDPPKNLQLKPLKNSRQVEVSWEYPDTWSTPHSYFSLTFCVQVQGKSKREKKDRVFTDKTSATVICRKNASISVRAQDRYYSSSWSEWASVPCSGSGSSRGGSGSGGSGGGGSRNLPVATPDPGMFPCLHHSQNLLRAVSNMLQKARQTLEFYPCTSEEIDHEDITKDKTSTVEACLPLELTKNESCLNSRETSFITNGSCLASRKTSFMMALCLSSIYEDLKMYQVEFKTMNAKLLMDPKRQIFLDQNMLAVIDELMQALNFNSETVPQKSSLEEPDFYKTKIKLCILLHAFRIRAVTIDRVMSYLNAS

SEQ ID NO: 10 - protein, 526 aa, Artificial sequence
MWELEKDVYVVEVDWTPDAPGETVNLTCDTPEEDDITWTSDQRHGVIGSGKTLTITVKEFLDAGQYTCHKGGETLSHSHLLLHKKENGIWSTEILKNFKNKTFLKCEAPNYSGRFTCSWLVQRNMDLKFNIKSSSSSPDSRAVTCGMASLSAEKVTLDQRDYEKYSVSCQEDVTCPTAEETLPIELALEARQQNKYENYSTSFFIRDIIKPDPPKNLQMKPLKNSQVEVSWEYPDSWSTPHSYFSLKFFVRIQRKKEKMKETEEGCNQKGAFLVEKTSTEVQCKGGNVCVQAQDRYYNSSCSKWACVPCRVRSGSGSSRGGSGSGGSGGGGSKRVIPVSGPARCLSQSRNLLKTTDDMVKTAREKLKHYSCTAEDIDHEDITRDQTSTLKTCLPLELHKNESCLATRETSSTTRGSCLPPQKTSLMMTLCLGSIYEDLKMYQTEFQAINAALQNHNHQQIILDKGMLVAIDELMQSLNHNGETLRQKPPVGEADPYRVKMKLCILLHAFSTRVVTINRVMGYLSSA

SEQ ID NO: 11 - protein, 114 aa, Artificial sequence
NWVNVISDLKKIEDLIQSMHIDATLYTESDVHPSCKVTAMKCFLLELQVISLESGDASIHDTVENLIILANDSLSSNGNVTESGCKECEELEEKNIKEFLQSFVHIVQMFINTS

SEQ ID NO: 12 - protein, 66 aa, Artificial sequence
ITCPPPMSVEHADIWVKSYSLYSRERYICNSGFKRKAGTSSLTECVLNKATNVAHWTTPSLKCIRD

SEQ ID NO: 13 - protein, 209 aa, Artificial sequence
ITCPPPMSVEHADIWVKSYSLYSRERYICNSGFKRKAGTSSLTECVLNKATNVAHWTTPSLKCIRGGGGSGGGGSGGGGSGGGGSGGGGSGGGGSNWVNVISDLKKIEDLIQSMHIDATLYTESDVHPSCKVTAMKCFLLELQVISLESGDASIHDTVENLIILANDSLSSNGNVTESGCKECEELEEKNIKEFLQSFVHIVQMFINTS

SEQ ID NO: 14 - protein, 232 aa, Artificial sequence
EPKSCDKTHTCPPCPAPELLGGPSVFLFPPKPKDTLMISRTPEVTCVVVDVSHEDPEVKFNWYVDGVEVHNAKTKPREEQYNSTYRVVSVLTVLHQDWLNGKEYKCKVSNKALPAPIEKTISKAKGQPREPQVYTLPPSREEMTKNQVSLTCLVKGFYPSDIAVEWESNGQPENNYKTTPPVLDSDGSFFLYSKLTVDKSRWQQGNVFSCSVMHEALHNHYTQKSLSLSPGK

SEQ ID NO: 15 - protein, 232 aa, Artificial sequence
EPKSCDKTHTCPPCPAPELLGGPSVFLFPPKPKDTLMISRTPEVTCVVVDVSHEDPEVKFNWYVDGVEVHNAKTKPREEQYNSTYRVVSVLTVLAQDWLNGKEYKCKVSNKALPAPIEKTISKAKGQPREPQVYTLPPSREEMTKNQVSLTCLVKGFYPSDIAVEWESNGQPENNYKTTPPVLDSDGSFFLYSKLTVDKSRWQQGNVFSCSVMHEALHNQYTQKSLSLSPGK

SEQ ID NO: 16 - protein, 229 aa, Artificial sequence
ESKYGPPCPPCPAPEFLGGPSVFLFPPKPKDTLMISRTPEVTCVVVDVSQEDPEVQFNWYVDGVEVHNAKTKPREEQFNSTYRVVSVLTVLHQDWLNGKEYKCKVSNKGLPSSIEKTISKAKGQPREPQVYTLPPSQEEMTKNQVSLTCLVKGFYPSDIAVEWESNGQPENNYKTTPPVLDSDGSFFLYSRLTVDKSRWQEGNVFSCSVMHEALHNHYTQKSLSLSLGK

SEQ ID NO: 17 - protein, 229 aa, Artificial sequence
ESKYGPPCPPCPAPEFLGGPSVFLFPPKPKDTLMISRTPEVTCVVVDVSQEDPEVQFNWYVDGVEVHNAKTKPREEQFNSTYRVVSVLTVLAQDWLNGKEYKCKVSNKGLPSSIEKTISKAKGQPREPQVYTLPPSQEEMTKNQVSLTCLVKGFYPSDIAVEWESNGQPENNYKTTPPVLDSDGSFFLYSRLTVDKSRWQEGNVFSCSVMHEALHNQYTQKSLSLSLGK

SEQ ID NO: 18 - protein, 362 aa, Artificial sequence
APTSSSTKKTQLQLEHLLLDLQMILNGINNYKNPKLTRMLTFKFYMPKKATELKHLQCLEEELKPLEEVLNLAQSKNFHLRPRDLISNINVIVLELKGSETTFMCEYADETATIVEFLNRWITFCQSIISTLTESKYGPPCPPCPAPEFLGGPSVFLFPPKPKDTLMISRTPEVTCVVVDVSQEDPEVQFNWYVDGVEVHNAKTKPREEQFNSTYRVVSVLTVLHQDWLNGKEYKCKVSNKGLPSSIEKTISKAKGQPREPQVYTLPPSQEEMTKNQVSLTCLVKGFYPSDIAVEWESNGQPENNYKTTPPVLDSDGSFFLYSRLTVDKSRWQEGNVFSCSVMHEALHNHYTQKSLSLSLGK

SEQ ID NO: 19 - protein, 362 aa, Artificial sequence
APTSSSTKKTQLQLEHLLLDLQMILNGINNYKNPKLTRMLTFKFYMPKKATELKHLQCLEEELKPLEEVLNLAQSKNFHLRPRDLISNINVIVLELKGSETTFMCEYADETATIVEFLNRWITFCQSIISTLTESKYGPPCPPCPAPEFLGGPSVFLFPPKPKDTLMISRTPEVTCVVVDVSQEDPEVQFNWYVDGVEVHNAKTKPREEQFNSTYRVVSVLTVLAQDWLNGKEYKCKVSNKGLPSSIEKTISKAKGQPREPQVYTLPPSQEEMTKNQVSLTCLVKGFYPSDIAVEWESNGQPENNYKTTPPVLDSDGSFFLYSRLTVDKSRWQEGNVFSCSVMHEALHNQYTQKSLSLSLGK

SEQ ID NO: 20 - protein, 754 aa, Artificial sequence
IWELKKDVYVVELDWYPDAPGEMVVLTCDTPEEDGITWTLDQSSEVLGSGKTLTIQVKEFGDAGQYTCHKGGEVLSHSLLLLHKKEDGIWSTDILKDQKEPKNKTFLRCEAKNYSGRFTCWWLTTISTDLTFSVKSSRGSSDPQGVTCGAATLSAERVRGDNKEYEYSVECQEDSACPAAEESLPIEVMVDAVHKLKYENYTSSFFIRDIIKPDPPKNLQLKPLKNSRQVEVSWEYPDTWSTPHSYFSLTFCVQVQGKSKREKKDRVFTDKTSATVICRKNASISVRAQDRYYSSSWSEWASVPCSGSGSSRGGSGSGGSGGGGSRNLPVATPDPGMFPCLHHSQNLLRAVSNMLQKARQTLEFYPCTSEEIDHEDITKDKTSTVEACLPLELTKNESCLNSRETSFITNGSCLASRKTSFMMALCLSSIYEDLKMYQVEFKTMNAKLLMDPKRQIFLDQNMLAVIDELMQALNFNSETVPQKSSLEEPDFYKTKIKLCILLHAFRIRAVTIDRVMSYLNASEPKSCDKTHTCPPCPAPELLGGPSVFLFPPKPKDTLMISRTPEVTCVVVDVSHEDPEVKFNWYVDGVEVHNAKTKPREEQYNSTYRVVSVLTVLHQDWLNGKEYKCKVSNKALPAPIEKTISKAKGQPREPQVYTLPPSRDELTKNQVSLTCLVKGFYPSDIAVEWESNGQPENNYKTTPPVLDSDGSFFLYSKLTVDKSRWQQGNVFSCSVMHEALHNHYTQKSLSLSPGK

SEQ ID NO: 21 - protein, 758 aa, Artificial sequence
MWELEKDVYVVEVDWTPDAPGETVNLTCDTPEEDDITWTSDQRHGVIGSGKTLTITVKEFLDAGQYTCHKGGETLSHSHLLLHKKENGIWSTEILKNFKNKTFLKCEAPNYSGRFTCSWLVQRNMDLKFNIKSSSSSPDSRAVTCGMASLSAEKVTLDQRDYEKYSVSCQEDVTCPTAEETLPIELALEARQQNKYENYSTSFFIRDIIKPDPPKNLQMKPLKNSQVEVSWEYPDSWSTPHSYFSLKFFVRIQRKKEKMKETEEGCNQKGAFLVEKTSTEVQCKGGNVCVQAQDRYYNSSCSKWACVPCRVRSGSGSSRGGSGSGGSGGGGSKRVIPVSGPARCLSQSRNLLKTTDDMVKTAREKLKHYSCTAEDIDHEDITRDQTSTLKTCLPLELHKNESCLATRETSSTTRGSCLPPQKTSLMMTLCLGSIYEDLKMYQTEFQAINAALQNHNHQQIILDKGMLVAIDELMQSLNHNGETLRQKPPVGEADPYRVKMKLCILLHAFSTRVVTINRVMGYLSSAEPKSCDKTHTCPPCPAPELLGGPSVFLFPPKPKDTLMISRTPEVTCVVVDVSHEDPEVKFNWYVDGVEVHNAKTKPREEQYNSTYRVVSVLTVLHQDWLNGKEYKCKVSNKALPAPIEKTISKAKGQPREPQVYTLPPSRDELTKNQVSLTCLVKGFYPSDIAVEWESNGQPENNYKTTPPVLDSDGSFFLYSKLTVDKSRWQQGNVFSCSVMHEALHNHYTQKSLSLSPGK

SEQ ID NO: 22 - protein, 754 aa, Artificial sequence
IWELKKDVYVVELDWYPDAPGEMVVLTCDTPEEDGITWTLDQSSEVLGSGKTLTIQVKEFGDAGQYTCHKGGEVLSHSLLLLHKKEDGIWSTDILKDQKEPKNKTFLRCEAKNYSGRFTCWWLTTISTDLTFSVKSSRGSSDPQGVTCGAATLSAERVRGDNKEYEYSVECQEDSACPAAEESLPIEVMVDAVHKLKYENYTSSFFIRDIIKPDPPKNLQLKPLKNSRQVEVSWEYPDTWSTPHSYFSLTFCVQVQGKSKREKKDRVFTDKTSATVICRKNASISVRAQDRYYSSSWSEWASVPCSGSGSSRGGSGSGGSGGGGSRNLPVATPDPGMFPCLHHSQNLLRAVSNMLQKARQTLEFYPCTSEEIDHEDITKDKTSTVEACLPLELTKNESCLNSRETSFITNGSCLASRKTSFMMALCLSSIYEDLKMYQVEFKTMNAKLLMDPKRQIFLDQNMLAVIDELMQALNFNSETVPQKSSLEEPDFYKTKIKLCILLHAFRIRAVTIDRVMSYLNASEPKSCDKTHTCPPCPAPELLGGPSVFLFPPKPKDTLMISRTPEVTCVVVDVSHEDPEVKFNWYVDGVEVHNAKTKPREEQYNSTYRVVSVLTVLAQDWLNGKEYKCKVSNKALPAPIEKTISKAKGQPREPQVYTLPPSRDELTKNQVSLTCLVKGFYPSDIAVEWESNGQPENNYKTTPPVLDSDGSFFLYSKLTVDKSRWQQGNVFSCSVMHEALHNQYTQKSLSLSPGK

SEQ ID NO: 23 - protein, 758 aa, Artificial sequence
MWELEKDVYVVEVDWTPDAPGETVNLTCDTPEEDDITWTSDQRHGVIGSGKTLTITVKEFLDAGQYTCHKGGETLSHSHLLLHKKENGIWSTEILKNFKNKTFLKCEAPNYSGRFTCSWLVQRNMDLKFNIKSSSSSPDSRAVTCGMASLSAEKVTLDQRDYEKYSVSCQEDVTCPTAEETLPIELALEARQQNKYENYSTSFFIRDIIKPDPPKNLQMKPLKNSQVEVSWEYPDSWSTPHSYFSLKFFVRIQRKKEKMKETEEGCNQKGAFLVEKTSTEVQCKGGNVCVQAQDRYYNSSCSKWACVPCRVRSGSGSSRGGSGSGGSGGGGSKRVIPVSGPARCLSQSRNLLKTTDDMVKTAREKLKHYSCTAEDIDHEDITRDQTSTLKTCLPLELHKNESCLATRETSSTTRGSCLPPQKTSLMMTLCLGSIYEDLKMYQTEFQAINAALQNHNHQQIILDKGMLVAIDELMQSLNHNGETLRQKPPVGEADPYRVKMKLCILLHAFSTRVVTINRVMGYLSSAEPKSCDKTHTCPPCPAPELLGGPSVFLFPPKPKDTLMISRTPEVTCVVVDVSHEDPEVKFNWYVDGVEVHNAKTKPREEQYNSTYRVVSVLTVLAQDWLNGKEYKCKVSNKALPAPIEKTISKAKGQPREPQVYTLPPSRDELTKNQVSLTCLVKGFYPSDIAVEWESNGQPENNYKTTPPVLDSDGSFFLYSKLTVDKSRWQQGNVFSCSVMHEALHNQYTQKSLSLSPGK

SEQ ID NO: 24 - protein, 441 aa, Artificial sequence
ITCPPPMSVEHADIWVKSYSLYSRERYICNSGFKRKAGTSSLTECVLNKATNVAHWTTPSLKCIRGGGGSGGGGSGGGGSGGGGSGGGGSGGGGSNWVNVISDLKKIEDLIQSMHIDATLYTESDVHPSCKVTAMKCFLLELQVISLESGDASIHDTVENLIILANDSLSSNGNVTESGCKECEELEEKNIKEFLQSFVHIVQMFINTSEPKSCDKTHTCPPCPAPELLGGPSVFLFPPKPKDTLMISRTPEVTCVVVDVSHEDPEVKFNWYVDGVEVHNAKTKPREEQYNSTYRVVSVLTVLHQDWLNGKEYKCKVSNKALPAPIEKTISKAKGQPREPQVYTLPPSREEMTKNQVSLTCLVKGFYPSDIAVEWESNGQPENNYKTTPPVLDSDGSFFLYSKLTVDKSRWQQGNVFSCSVMHEALHNHYTQKSLSLSPGK

SEQ ID NO: 25 - protein, 441 aa, Artificial sequence
ITCPPPMSVEHADIWVKSYSLYSRERYICNSGFKRKAGTSSLTECVLNKATNVAHWTTPSLKCIRGGGGSGGGGSGGGGSGGGGSGGGGSGGGGSNWVNVISDLKKIEDLIQSMHIDATLYTESDVHPSCKVTAMKCFLLELQVISLESGDASIHDTVENLIILANDSLSSNGNVTESGCKECEELEEKNIKEFLQSFVHIVQMFINTSEPKSCDKTHTCPPCPAPELLGGPSVFLFPPKPKDTLMISRTPEVTCVVVDVSHEDPEVKFNWYVDGVEVHNAKTKPREEQYNSTYRVVSVLTVLAQDWLNGKEYKCKVSNKALPAPIEKTISKAKGQPREPQVYTLPPSREEMTKNQVSLTCLVKGFYPSDIAVEWESNGQPENNYKTTPPVLDSDGSFFLYSKLTVDKSRWQQGNVFSCSVMHEALHNQYTQKSLSLSPGK

SEQ ID NO: 26 - protein, 444 aa, Artificial sequence
QVQLVQSGAEVKKPGASVKVSCKASGFNIKNTYMHWVRQAPGQGLEWMGRIDPANGNTKYAPKFQGRVTMTRDTSTSTVYMELSSLRSEDTAVYYCGRSRGYAMDYWGQGTTVTVSSASTKGPSVFPLAPCSRSTSESTAALGCLVKDYFPEPVTVSWNSGALTSGVHTFPAVLQSSGLYSLSSVVTVPSSSLGTKTYTCNVDHKPSNTKVDKRVESKYGPPCPPCPAPEFLGGPSVFLFPPKPKDTLMISRTPEVTCVVVDVSQEDPEVQFNWYVDGVEVHNAKTKPREEQFNSTYRVVSVLTVLAQDWLNGKEYKCKVSNKGLPSSIEKTISKAKGQPREPQVYTLPPSQEEMTKNQVSLTCLVKGFYPSDIAVEWESNGQPENNYKTTPPVLDSDGSFFLYSRLTVDKSRWQEGNVFSCSVMHEALHNQYTQKSLSLSLGK

SEQ ID NO: 27 - protein, 444 aa, Artificial sequence
QVQLVQSGAEVKKPGASVKVSCKASGFNIKNTYMHWVRQAPGQGLEWMGRIDPANGNTKYAPKFQGRVTMTRDTSTSTVYMELSSLRSEDTAVYYCGRSRGYAMDYWGQGTTVTVSSASTKGPSVFPLAPCSRSTSESTAALGCLVKDYFPEPVTVSWNSGALTSGVHTFPAVLQSSGLYSLSSVVTVPSSSLGTKTYTCNVDHKPSNTKVDKRVESKYGPPCPPCPAPEFLGGPSVFLFPPKPKDTLMISRTPEVTCVVVDVSQEDPEVQFNWYVDGVEVHNAKTKPREEQFNSTYRVVSVLTVLHQDWLNGKEYKCKVSNKGLPSSIEKTISKAKGQPREPQVYTLPPSQEEMTKNQVSLTCLVKGFYPSDIAVEWESNGQPENNYKTTPPVLDSDGSFFLYSRLTVDKSRWQEGNVFSCSVMHEALHNHYTQKSLSLSLGK

SEQ ID NO: 28 - protein, 213 aa, Artificial sequence
DIQMTQSPSSLSASVGDRVTITCKASDHINNWLAWYQQKPGKAPKLLISGATSLETGVPSRFSGSGSGTDYTLTISSLQPEDFATYYCQQYWSTPTFGGGTKLEIKRTVAAPSVFIFPPSDEQLKSGTASVVCLLNNFYPREAKVQWKVDNALQSGNSQESVTEQDSKDSTYSLSSTLTLSKADYEKHKVYACEVTHQGLSSPVTKSFNRGEC

SEQ ID NO: 29 - protein, 452 aa, Artificial sequence
QVQLVQSGAEVKKPGSSVKVSCKASGYIFTADWIYWVRQAPGQGLEWMGRIYPGVDTTYYAQKFQGRVTITADKSTSTAYMELSSLRSEDTAVYYCARGGEVRRDFYALDYWGQGTTVTVSSASTKGPSVFPLAPSSKSTSGGTAALGCLVKDYFPEPVTVSWNSGALTSGVHTFPAVLQSSGLYSLSSVVTVPSSSLGTQTYICNVNHKPSNTKVDKKVEPKSCDKTHTCPPCPAPELLGGPSVFLFPPKPKDTLMISRTPEVTCVVVDVSHEDPEVKFNWYVDGVEVHNAKTKPREEQYNSTYRVVSVLTVLHQDWLNGKEYKCKVSNKALPAPIEKTISKAKGQPREPQVYTLPPSRDELTKNQVSLTCLVKGFYPSDIAVEWESNGQPENNYKTTPPVLDSDGSFFLYSKLTVDKSRWQQGNVFSCSVMHEALHNHYTQKSLSLSPGK

SEQ ID NO: 30 - protein, 676 aa, Artificial sequence
QVQLVQSGAEVKKPGSSVKVSCKASGYIFTADWIYWVRQAPGQGLEWMGRIYPGVDTTYYAQKFQGRVTITADKSTSTAYMELSSLRSEDTAVYYCARGGEVRRDFYALDYWGQGTTVTVSSASTKGPSVFPLAPSSKSTSGGTAALGCLVKDYFPEPVTVSWNSGALTSGVHTFPAVLQSSGLYSLSSVVTVPSSSLGTQTYICNVNHKPSNTKVDKKVEPKSCDKTHTCPPCPAPELLGGPSVFLFPPKPKDTLMISRTPEVTCVVVDVSHEDPEVKFNWYVDGVEVHNAKTKPREEQYNSTYRVVSVLTVLHQDWLNGKEYKCKVSNKALPAPIEKTISKAKGQPREPQVYTLPPSRDELTKNQVSLTCLVKGFYPSDIAVEWESNGQPENNYKTTPPVLDSDGSFFLYSKLTVDKSRWQQGNVFSCSVMHEALHNHYTQKSLSLSPGKGGGGSGGGGSGGGGSITCPPPMSVEHADIWVKSYSLYSRERYICNSGFKRKAGTSSLTECVLNKATNVAHWTTPSLKCIRGGGGSGGGGSGGGGSGGGGSGGGGSGGGGSNWVNVISDLKKIEDLIQSMHIDATLYTESDVHPSCKVTAMKCFLLELQVISLESGDASIHDTVENLIILANDSLSSNGNVTESGCKECEELEEKNIKEFLQSFVHIVQMFINTS

SEQ ID NO: 31 - protein, 452 aa, Artificial sequence
QVQLVQSGAEVKKPGSSVKVSCKASGYIFTADWIYWVRQAPGQGLEWMGRIYPGVDTTYYAQKFQGRVTITADKSTSTAYMELSSLRSEDTAVYYCARGGEVRRDFYALDYWGQGTTVTVSSASTKGPSVFPLAPSSKSTSGGTAALGCLVKDYFPEPVTVSWNSGALTSGVHTFPAVLQSSGLYSLSSVVTVPSSSLGTQTYICNVNHKPSNTKVDKKVEPKSCDKTHTCPPCPAPELLGGPSVFLFPPKPKDTLMISRTPEVTCVVVDVSHEDPEVKFNWYVDGVEVHNAKTKPREEQYNSTYRVVSVLTVLAQDWLNGKEYKCKVSNKALPAPIEKTISKAKGQPREPQVYTLPPSRDELTKNQVSLTCLVKGFYPSDIAVEWESNGQPENNYKTTPPVLDSDGSFFLYSKLTVDKSRWQQGNVFSCSVMHEALHNQYTQKSLSLSPGK

SEQ ID NO: 32 - protein, 676 aa, Artificial sequence
QVQLVQSGAEVKKPGSSVKVSCKASGYIFTADWIYWVRQAPGQGLEWMGRIYPGVDTTYYAQKFQGRVTITADKSTSTAYMELSSLRSEDTAVYYCARGGEVRRDFYALDYWGQGTTVTVSSASTKGPSVFPLAPSSKSTSGGTAALGCLVKDYFPEPVTVSWNSGALTSGVHTFPAVLQSSGLYSLSSVVTVPSSSLGTQTYICNVNHKPSNTKVDKKVEPKSCDKTHTCPPCPAPELLGGPSVFLFPPKPKDTLMISRTPEVTCVVVDVSHEDPEVKFNWYVDGVEVHNAKTKPREEQYNSTYRVVSVLTVLAQDWLNGKEYKCKVSNKALPAPIEKTISKAKGQPREPQVYTLPPSRDELTKNQVSLTCLVKGFYPSDIAVEWESNGQPENNYKTTPPVLDSDGSFFLYSKLTVDKSRWQQGNVFSCSVMHEALHNQYTQKSLSLSPGKGGGGSGGGGSGGGGSITCPPPMSVEHADIWVKSYSLYSRERYICNSGFKRKAGTSSLTECVLNKATNVAHWTTPSLKCIRGGGGSGGGGSGGGGSGGGGSGGGGSGGGGSNWVNVISDLKKIEDLIQSMHIDATLYTESDVHPSCKVTAMKCFLLELQVISLESGDASIHDTVENLIILANDSLSSNGNVTESGCKECEELEEKNIKEFLQSFVHIVQMFINTS

SEQ ID NO: 33 - protein, 214 aa, Artificial sequence
EIVLTQSPATLSLSPGERATLSCRASENVGTYVSWYQQKPGQAPRLLIYGASNRYTGIPARFSGSGSGTDFTLTISSLEPEDFAVYYCGQRYSYPFTFGGGTKLEIKRTVAAPSVFIFPPSDEQLKSGTASVVCLLNNFYPREAKVQWKVDNALQSGNSQESVTEQDSKDSTYSLSSTLTLSKADYEKHKVYACEVTHQGLSSPVTKSFNRGEC

SEQ ID NO: 34 - protein, 452 aa, Artificial sequence
QVQLVQSGAEVKKPGASVKVSCKASGYTFTSYWMYWVRQAPGQRLEWIGTIYPGNSDTNYSQKFQGRVTITADTSASTAYMELSSLRSEDTAVYYCTREGSKGYDVWYFAVWGQGTTVTVSSASTKGPSVFPLAPSSKSTSGGTAALGCLVKDYFPEPVTVSWNSGALTSGVHTFPAVLQSSGLYSLSSVVTVPSSSLGTQTYICNVNHKPSNTKVDKKVEPKSCDKTHTCPPCPAPELLGGPSVFLFPPKPKDTLMISRTPEVTCVVVDVSHEDPEVKFNWYVDGVEVHNAKTKPREEQYNSTYRVVSVLTVLHQDWLNGKEYKCKVSNKALPAPIEKTISKAKGQPREPQVYTLPPSRDELTKNQVSLTCLVKGFYPSDIAVEWESNGQPENNYKTTPPVLDSDGSFFLYSKLTVDKSRWQQGNVFSCSVMHEALHNHYTQKSLSLSPGK

SEQ ID NO: 35 - protein, 676 aa, Artificial sequence
QVQLVQSGAEVKKPGASVKVSCKASGYTFTSYWMYWVRQAPGQRLEWIGTIYPGNSDTNYSQKFQGRVTITADTSASTAYMELSSLRSEDTAVYYCTREGSKGYDVWYFAVWGQGTTVTVSSASTKGPSVFPLAPSSKSTSGGTAALGCLVKDYFPEPVTVSWNSGALTSGVHTFPAVLQSSGLYSLSSVVTVPSSSLGTQTYICNVNHKPSNTKVDKKVEPKSCDKTHTCPPCPAPELLGGPSVFLFPPKPKDTLMISRTPEVTCVVVDVSHEDPEVKFNWYVDGVEVHNAKTKPREEQYNSTYRVVSVLTVLHQDWLNGKEYKCKVSNKALPAPIEKTISKAKGQPREPQVYTLPPSRDELTKNQVSLTCLVKGFYPSDIAVEWESNGQPENNYKTTPPVLDSDGSFFLYSKLTVDKSRWQQGNVFSCSVMHEALHNHYTQKSLSLSPGKGGGGSGGGGSGGGGSITCPPPMSVEHADIWVKSYSLYSRERYICNSGFKRKAGTSSLTECVLNKATNVAHWTTPSLKCIRGGGGSGGGGSGGGGSGGGGSGGGGSGGGGSNWVNVISDLKKIEDLIQSMHIDATLYTESDVHPSCKVTAMKCFLLELQVISLESGDASIHDTVENLIILANDSLSSNGNVTESGCKECEELEEKNIKEFLQSFVHIVQMFINTS

SEQ ID NO: 36 - protein, 452 aa, Artificial sequence
QVQLVQSGAEVKKPGASVKVSCKASGYTFTSYWMYWVRQAPGQRLEWIGTIYPGNSDTNYSQKFQGRVTITADTSASTAYMELSSLRSEDTAVYYCTREGSKGYDVWYFAVWGQGTTVTVSSASTKGPSVFPLAPSSKSTSGGTAALGCLVKDYFPEPVTVSWNSGALTSGVHTFPAVLQSSGLYSLSSVVTVPSSSLGTQTYICNVNHKPSNTKVDKKVEPKSCDKTHTCPPCPAPELLGGPSVFLFPPKPKDTLMISRTPEVTCVVVDVSHEDPEVKFNWYVDGVEVHNAKTKPREEQYNSTYRVVSVLTVLAQDWLNGKEYKCKVSNKALPAPIEKTISKAKGQPREPQVYTLPPSRDELTKNQVSLTCLVKGFYPSDIAVEWESNGQPENNYKTTPPVLDSDGSFFLYSKLTVDKSRWQQGNVFSCSVMHEALHNQYTQKSLSLSPGK

SEQ ID NO: 37 - protein, 676 aa, Artificial sequence
QVQLVQSGAEVKKPGASVKVSCKASGYTFTSYWMYWVRQAPGQRLEWIGTIYPGNSDTNYSQKFQGRVTITADTSASTAYMELSSLRSEDTAVYYCTREGSKGYDVWYFAVWGQGTTVTVSSASTKGPSVFPLAPSSKSTSGGTAALGCLVKDYFPEPVTVSWNSGALTSGVHTFPAVLQSSGLYSLSSVVTVPSSSLGTQTYICNVNHKPSNTKVDKKVEPKSCDKTHTCPPCPAPELLGGPSVFLFPPKPKDTLMISRTPEVTCVVVDVSHEDPEVKFNWYVDGVEVHNAKTKPREEQYNSTYRVVSVLTVLAQDWLNGKEYKCKVSNKALPAPIEKTISKAKGQPREPQVYTLPPSRDELTKNQVSLTCLVKGFYPSDIAVEWESNGQPENNYKTTPPVLDSDGSFFLYSKLTVDKSRWQQGNVFSCSVMHEALHNQYTQKSLSLSPGKGGGGSGGGGSGGGGSITCPPPMSVEHADIWVKSYSLYSRERYICNSGFKRKAGTSSLTECVLNKATNVAHWTTPSLKCIRGGGGSGGGGSGGGGSGGGGSGGGGSGGGGSNWVNVISDLKKIEDLIQSMHIDATLYTESDVHPSCKVTAMKCFLLELQVISLESGDASIHDTVENLIILANDSLSSNGNVTESGCKECEELEEKNIKEFLQSFVHIVQMFINTS

SEQ ID NO: 38 - protein, 218 aa, Artificial sequence
DIQMTQSPSSLSASVGDRVTITCRASKSVSTSGYSYMHWYQQKPGKAPKLLIYLASNLESGVPSRFSGSGSGTDFTLTISSLQPEDFATYYCQHSRELPFTFGGGTKLEIKRTVAAPSVFIFPPSDEQLKSGTASVVCLLNNFYPREAKVQWKVDNALQSGNSQESVTEQDSKDSTYSLSSTLTLSKADYEKHKVYACEVTHQGLSSPVTKSFNRGEC

SEQ ID NO: 39 - protein, 447 aa, Artificial sequence
QVQLVQSGAEVKKPGASVKVSCKGSGYTFTDYAIHWVRQAPGQSLEWIGVFSIYYENINYNQKFKGRATMTVDKSTSTAYMELRSLRSDDTAVYYCARRDGGTINYWGQGTLVTVSSASTKGPSVFPLAPSSKSTSGGTAALGCLVKDYFPEPVTVSWNSGALTSGVHTFPAVLQSSGLYSLSSVVTVPSSSLGTQTYICNVNHKPSNTKVDKKVEPKSCDKTHTCPPCPAPELLGGPSVFLFPPKPKDTLMISRTPEVTCVVVDVSHEDPEVKFNWYVDGVEVHNAKTKPREEQYNSTYRVVSVLTVLHQDWLNGKEYKCKVSNKALPAPIEKTISKAKGQPREPQVYTLPPSREEMTKNQVSLTCLVKGFYPSDIAVEWESNGQPENNYKTTPPVLDSDGSFFLYSKLTVDKSRWQQGNVFSCSVMHEALHNHYTQKSLSLSPGK

SEQ ID NO: 40 - protein, 671 aa, Artificial sequence
QVQLVQSGAEVKKPGASVKVSCKGSGYTFTDYAIHWVRQAPGQSLEWIGVFSIYYENINYNQKFKGRATMTVDKSTSTAYMELRSLRSDDTAVYYCARRDGGTINYWGQGTLVTVSSASTKGPSVFPLAPSSKSTSGGTAALGCLVKDYFPEPVTVSWNSGALTSGVHTFPAVLQSSGLYSLSSVVTVPSSSLGTQTYICNVNHKPSNTKVDKKVEPKSCDKTHTCPPCPAPELLGGPSVFLFPPKPKDTLMISRTPEVTCVVVDVSHEDPEVKFNWYVDGVEVHNAKTKPREEQYNSTYRVVSVLTVLHQDWLNGKEYKCKVSNKALPAPIEKTISKAKGQPREPQVYTLPPSREEMTKNQVSLTCLVKGFYPSDIAVEWESNGQPENNYKTTPPVLDSDGSFFLYSKLTVDKSRWQQGNVFSCSVMHEALHNHYTQKSLSLSPGKGGGGSGGGGSGGGGSITCPPPMSVEHADIWVKSYSLYSRERYICNSGFKRKAGTSSLTECVLNKATNVAHWTTPSLKCIRGGGGSGGGGSGGGGSGGGGSGGGGSGGGGSNWVNVISDLKKIEDLIQSMHIDATLYTESDVHPSCKVTAMKCFLLELQVISLESGDASIHDTVENLIILANDSLSSNGNVTESGCKECEELEEKNIKEFLQSFVHIVQMFINTS

SEQ ID NO: 41 - protein, 447 aa, Artificial sequence
QVQLVQSGAEVKKPGASVKVSCKGSGYTFTDYAIHWVRQAPGQSLEWIGVFSIYYENINYNQKFKGRATMTVDKSTSTAYMELRSLRSDDTAVYYCARRDGGTINYWGQGTLVTVSSASTKGPSVFPLAPSSKSTSGGTAALGCLVKDYFPEPVTVSWNSGALTSGVHTFPAVLQSSGLYSLSSVVTVPSSSLGTQTYICNVNHKPSNTKVDKKVEPKSCDKTHTCPPCPAPELLGGPSVFLFPPKPKDTLMISRTPEVTCVVVDVSHEDPEVKFNWYVDGVEVHNAKTKPREEQYNSTYRVVSVLTVLAQDWLNGKEYKCKVSNKALPAPIEKTISKAKGQPREPQVYTLPPSREEMTKNQVSLTCLVKGFYPSDIAVEWESNGQPENNYKTTPPVLDSDGSFFLYSKLTVDKSRWQQGNVFSCSVMHEALHNQYTQKSLSLSPGK

SEQ ID NO: 42 - protein, 671 aa, Artificial sequence
QVQLVQSGAEVKKPGASVKVSCKGSGYTFTDYAIHWVRQAPGQSLEWIGVFSIYYENINYNQKFKGRATMTVDKSTSTAYMELRSLRSDDTAVYYCARRDGGTINYWGQGTLVTVSSASTKGPSVFPLAPSSKSTSGGTAALGCLVKDYFPEPVTVSWNSGALTSGVHTFPAVLQSSGLYSLSSVVTVPSSSLGTQTYICNVNHKPSNTKVDKKVEPKSCDKTHTCPPCPAPELLGGPSVFLFPPKPKDTLMISRTPEVTCVVVDVSHEDPEVKFNWYVDGVEVHNAKTKPREEQYNSTYRVVSVLTVLAQDWLNGKEYKCKVSNKALPAPIEKTISKAKGQPREPQVYTLPPSREEMTKNQVSLTCLVKGFYPSDIAVEWESNGQPENNYKTTPPVLDSDGSFFLYSKLTVDKSRWQQGNVFSCSVMHEALHNQYTQKSLSLSPGKGGGGSGGGGSGGGGSITCPPPMSVEHADIWVKSYSLYSRERYICNSGFKRKAGTSSLTECVLNKATNVAHWTTPSLKCIRGGGGSGGGGSGGGGSGGGGSGGGGSGGGGSNWVNVISDLKKIEDLIQSMHIDATLYTESDVHPSCKVTAMKCFLLELQVISLESGDASIHDTVENLIILANDSLSSNGNVTESGCKECEELEEKNIKEFLQSFVHIVQMFINTS

SEQ ID NO: 43 - protein, 219 aa, Artificial sequence
DVVMTQSPLSLPVTLGQPASISCRSSQSLVHSNGNTYLHWYQQRPGQSPRLLIYKVSNRFSGVPDRFSGSGSGTDFTLKISRVEAEDVGVYFCSQSTHIPWTFGQGTKVEIKRTVAAPSVFIFPPSDEQLKSGTASVVCLLNNFYPREAKVQWKVDNALQSGNSQESVTEQDSKDSTYSLSSTLTLSKADYEKHKVYACEVTHQGLSSPVTKSFNRGEC

SEQ ID NO: 44 - protein, 668 aa, Artificial sequence
EVKLVESGGGLVQPGGSLRLSCAASGFAFSSYDMSWVRQAPGKRLEWVATISGGGRYTYYPDTVKGRFTISRDNAKNSHYLQMNSLRAEDTAVYFCASPYGGYFDVWGQGTLVTVSSASTKGPSVFPLAPCSRSTSESTAALGCLVKDYFPEPVTVSWNSGALTSGVHTFPAVLQSSGLYSLSSVVTVPSSSLGTKTYTCNVDHKPSNTKVDKRVESKYGPPCPPCPAPEFLGGPSVFLFPPKPKDTLMISRTPEVTCVVVDVSQEDPEVQFNWYVDGVEVHNAKTKPREEQFNSTYRVVSVLTVLHQDWLNGKEYKCKVSNKGLPSSIEKTISKAKGQPREPQVYTLPPSQEEMTKNQVSLTCLVKGFYPSDIAVEWESNGQPENNYKTTPPVLDSDGSFFLYSRLTVDKSRWQEGNVFSCSVMHEALHNHYTQKSLSLSLGKGGGGSGGGGSGGGGSITCPPPMSVEHADIWVKSYSLYSRERYICNSGFKRKAGTSSLTECVLNKATNVAHWTTPSLKCIRGGGGSGGGGSGGGGSGGGGSGGGGSGGGGSNWVNVISDLKKIEDLIQSMHIDATLYTESDVHPSCKVTAMKCFLLELQVISLESGDASIHDTVENLIILANDSLSSNGNVTESGCKECEELEEKNIKEFLQSFVHIVQMFINTS

SEQ ID NO: 45 - protein, 668 aa, Artificial sequence; identical to SEQ ID NO: 44

SEQ ID NO: 46 - protein, 444 aa, Artificial sequence
EVKLVESGGGLVQPGGSLRLSCAASGFAFSSYDMSWVRQAPGKRLEWVATISGGGRYTYYPDTVKGRFTISRDNAKNSHYLQMNSLRAEDTAVYFCASPYGGYFDVWGQGTLVTVSSASTKGPSVFPLAPCSRSTSESTAALGCLVKDYFPEPVTVSWNSGALTSGVHTFPAVLQSSGLYSLSSVVTVPSSSLGTKTYTCNVDHKPSNTKVDKRVESKYGPPCPPCPAPEFLGGPSVFLFPPKPKDTLMISRTPEVTCVVVDVSQEDPEVQFNWYVDGVEVHNAKTKPREEQFNSTYRVVSVLTVLAQDWLNGKEYKCKVSNKGLPSSIEKTISKAKGQPREPQVYTLPPSQEEMTKNQVSLTCLVKGFYPSDIAVEWESNGQPENNYKTTPPVLDSDGSFFLYSRLTVDKSRWQEGNVFSCSVMHEALHNQYTQKSLSLSLGK

SEQ ID NO: 47 - protein, 668 aa, Artificial sequence
EVKLVESGGGLVQPGGSLRLSCAASGFAFSSYDMSWVRQAPGKRLEWVATISGGGRYTYYPDTVKGRFTISRDNAKNSHYLQMNSLRAEDTAVYFCASPYGGYFDVWGQGTLVTVSSASTKGPSVFPLAPCSRSTSESTAALGCLVKDYFPEPVTVSWNSGALTSGVHTFPAVLQSSGLYSLSSVVTVPSSSLGTKTYTCNVDHKPSNTKVDKRVESKYGPPCPPCPAPEFLGGPSVFLFPPKPKDTLMISRTPEVTCVVVDVSQEDPEVQFNWYVDGVEVHNAKTKPREEQFNSTYRVVSVLTVLAQDWLNGKEYKCKVSNKGLPSSIEKTISKAKGQPREPQVYTLPPSQEEMTKNQVSLTCLVKGFYPSDIAVEWESNGQPENNYKTTPPVLDSDGSFFLYSRLTVDKSRWQEGNVFSCSVMHEALHNQYTQKSLSLSLGKGGGGSGGGGSGGGGSITCPPPMSVEHADIWVKSYSLYSRERYICNSGFKRKAGTSSLTECVLNKATNVAHWTTPSLKCIRGGGGSGGGGSGGGGSGGGGSGGGGSGGGGSNWVNVISDLKKIEDLIQSMHIDATLYTESDVHPSCKVTAMKCFLLELQVISLESGDASIHDTVENLIILANDSLSSNGNVTESGCKECEELEEKNIKEFLQSFVHIVQMFINTS

SEQ ID NO: 48 - protein, 214 aa, Artificial sequence
EIVLTQSPATLSLSPGERATLSCRASQSISNFLHWYQQKPGQAPRLLIKYASQSISGIPARFSGSGSGTDFTLTISSLEPEDFAVYFCQQSNSWPHTFGQGTKVEIKRTVAAPSVFIFPPSDEQLKSGTASVVCLLNNFYPREAKVQWKVDNALQSGNSQESVTEQDSKDSTYSLSSTLTLSKADYEKHKVYACEVTHQGLSSPVTKSFNRGEC

SEQ ID NO: 49 - protein, 448 aa, Artificial sequence
QVQLQQSGAELVKPGASVRLSCKASGYTFTNYYIYWVRQRPGQGLEWIGEINPSNGGTHFNEKFKSKATVTVDKSSSTAYMQLSSLTSEDSAVYYCTRDLGYYAMDYWGQGTSVTVSSASTKGPSVFPLAPSSKSTSGGTAALGCLVKDYFPEPVTVSWNSGALTSGVHTFPAVLQSSGLYSLSSVVTVPSSSLGTQTYICNVNHKPSNTKVDKKVEPKSCDKTHTCPPCPAPELLGGPSVFLFPPKPKDTLMISRTPEVTCVVVDVSHEDPEVKFNWYVDGVEVHNAKTKPREEQYNSTYRVVSVLTVLHQDWLNGKEYKCKVSNKALPAPIEKTISKAKGQPREPQVYTLPPSREEMTKNQVSLTCLVKGFYPSDIAVEWESNGQPENNYKTTPPVLDSDGSFFLYSKLTVDKSRWQQGNVFSCSVMHEALHNHYTQKSLSLSPGK

SEQ ID NO: 50 - protein, 672 aa, Artificial sequence
QVQLQQSGAELVKPGASVRLSCKASGYTFTNYYIYWVRQRPGQGLEWIGEINPSNGGTHFNEKFKSKATVTVDKSSSTAYMQLSSLTSEDSAVYYCTRDLGYYAMDYWGQGTSVTVSSASTKGPSVFPLAPSSKSTSGGTAALGCLVKDYFPEPVTVSWNSGALTSGVHTFPAVLQSSGLYSLSSVVTVPSSSLGTQTYICNVNHKPSNTKVDKKVEPKSCDKTHTCPPCPAPELLGGPSVFLFPPKPKDTLMISRTPEVTCVVVDVSHEDPEVKFNWYVDGVEVHNAKTKPREEQYNSTYRVVSVLTVLHQDWLNGKEYKCKVSNKALPAPIEKTISKAKGQPREPQVYTLPPSREEMTKNQVSLTCLVKGFYPSDIAVEWESNGQPENNYKTTPPVLDSDGSFFLYSKLTVDKSRWQQGNVFSCSVMHEALHNHYTQKSLSLSPGKGGGGSGGGGSGGGGSITCPPPMSVEHADIWVKSYSLYSRERYICNSGFKRKAGTSSLTECVLNKATNVAHWTTPSLKCIRGGGGSGGGGSGGGGSGGGGSGGGGSGGGGSNWVNVISDLKKIEDLIQSMHIDATLYTESDVHPSCKVTAMKCFLLELQVISLESGDASIHDTVENLIILANDSLSSNGNVTESGCKECEELEEKNIKEFLQSFVHIVQMFINTS

SEQ ID NO: 51 - protein, 446 aa, Artificial sequence
QVQLQQSGAELVKPGASVRLSCKASGYTFTNYYIYWVRQRPGQGLEWIGEINPSNGGTHFNEKFKSKATVTVDKSSSTAYMQLSSLTSEDSAVYYCTRDLGYYAMDYWGQGTSVTVSSASTKGPSVFPLAPCSRSTSESTAALGCLVKDYFPEPVTVSWNSGALTSGVHTFPAVLQSSGLYSLSSVVTVPSSSLGTKTYTCNVDHKPSNTKVDKRVESKYGPPCPPCPAPEFLGGPSVFLFPPKPKDTLMISRTPEVTCVVVDVSQEDPEVQFNWYVDGVEVHNAKTKPREEQFNSTYRVVSVLTVLAQDWLNGKEYKCKVSNKGLPSSIEKTISKAKGQPREPQVYTLPPSQEEMTKNQVSLTCLVKGFYPSDIAVEWESNGQPENNYKTTPPVLDSDGSFFLYSRLTVDKSRWQEGNVFSCSVMHEALHNQYTQKSLSLSLGKG

SEQ ID NO: 52 - protein, 669 aa, Artificial sequence
QVQLQQSGAELVKPGASVRLSCKASGYTFTNYYIYWVRQRPGQGLEWIGEINPSNGGTHFNEKFKSKATVTVDKSSSTAYMQLSSLTSEDSAVYYCTRDLGYYAMDYWGQGTSVTVSSASTKGPSVFPLAPCSRSTSESTAALGCLVKDYFPEPVTVSWNSGALTSGVHTFPAVLQSSGLYSLSSVVTVPSSSLGTKTYTCNVDHKPSNTKVDKRVESKYGPPCPPCPAPEFLGGPSVFLFPPKPKDTLMISRTPEVTCVVVDVSQEDPEVQFNWYVDGVEVHNAKTKPREEQFNSTYRVVSVLTVLAQDWLNGKEYKCKVSNKGLPSSIEKTISKAKGQPREPQVYTLPPSQEEMTKNQVSLTCLVKGFYPSDIAVEWESNGQPENNYKTTPPVLDSDGSFFLYSRLTVDKSRWQEGNVFSCSVMHEALHNQYTQKSLSLSLGKGGGGSGGGGSGGGGSITCPPPMSVEHADIWVKSYSLYSRERYICNSGFKRKAGTSSLTECVLNKATNVAHWTTPSLKCIRGGGGSGGGGSGGGGSGGGGSGGGGSGGGGSNWVNVISDLKKIEDLIQSMHIDATLYTESDVHPSCKVTAMKCFLLELQVISLESGDASIHDTVENLIILANDSLSSNGNVTESGCKECEELEEKNIKEFLQSFVHIVQMFINTS

SEQ ID NO: 53 - protein, 214 aa, Artificial sequence
DIQMTQTTSSLSASLGDRVTISCRASQDIKNYLNWYQQRPDGTVNLLIYYTSRLQSGVPSRFSGSGSGTDYSLTINNLEQEDIATYFCQQGETLPWTFGGGTKLEIKRTVAAPSVFIFPPSDEQLKSGTASVVCLLNNFYPREAKVQWKVDNALQSGNSQESVTEQDSKDSTYSLSSTLTLSKADYEKHKVYACEVTHQGLSSPVTKSFNRGEC

SEQ ID NO: 54 - protein, 451 aa, Artificial sequence
QVQLQQPGAELVKPGASVKMSCKASGYTFTSYNMHWVKQTPGRGLEWIGAIYPGNGDTSYNQKFKGKATLTADKSSSTAYMQLSSLTSEDSAVYYCARSTYYGGDWYFNVWGAGTTVTVSAASTKGPSVFPLAPSSKSTSGGTAALGCLVKDYFPEPVTVSWNSGALTSGVHTFPAVLQSSGLYSLSSVVTVPSSSLGTQTYICNVNHKPSNTKVDKKAEPKSCDKTHTCPPCPAPELLGGPSVFLFPPKPKDTLMISRTPEVTCVVVDVSHEDPEVKFNWYVDGVEVHNAKTKPREEQYNSTYRVVSVLTVLAQDWLNGKEYKCKVSNKALPAPIEKTISKAKGQPREPQVYTLPPSRDELTKNQVSLTCLVKGFYPSDIAVEWESNGQPENNYKTTPPVLDSDGSFFLYSKLTVDKSRWQQGNVFSCSVMHEALHNQYTQKSLSLSPGK

SEQ ID NO: 55 - protein, 213 aa, Artificial sequence
QIVLSQSPAILSASPGEKVTMTCRASSSVSYIHWFQQKPGSSPKPWIYATSNLASGVPVRFSGSGSGTSYSLTISRVEAEDAATYYCQQWTSNPPTFGGGTKLEIKRTVAAPSVFIFPPSDEQLKSGTASVVCLLNNFYPREAKVQWKVDNALQSGNSQESVTEQDSKDSTYSLSSTLTLSKADYEKHKVYACEVTHQGLSSPVTKSFNRGEC

SEQ ID NO: 56 - protein, 449 aa, Artificial sequence
QVQLKQSGPGLVQPSQSLSITCTVSGFSLTNYGVHWVRQSPGKGLEWLGVIWSGGNTDYNTPFTSRLSINKDNSKSQVFFKMNSLQSNDTAIYYCARALTYYDYEFAYWGQGTLVTVSAASTKGPSVFPLAPSSKSTSGGTAALGCLVKDYFPEPVTVSWNSGALTSGVHTFPAVLQSSGLYSLSSVVTVPSSSLGTQTYICNVNHKPSNTKVDKKVEPKSCDKTHTCPPCPAPELLGGPSVFLFPPKPKDTLMISRTPEVTCVVVDVSHEDPEVKFNWYVDGVEVHNAKTKPREEQYNSTYRVVSVLTVLAQDWLNGKEYKCKVSNKALPAPIEKTISKAKGQPREPQVYTLPPSRDELTKNQVSLTCLVKGFYPSDIAVEWESNGQPENNYKTTPPVLDSDGSFFLYSKLTVDKSRWQQGNVFSCSVMHEALHNQYTQKSLSLSPGK

SEQ ID NO: 57 - protein, 214 aa, Artificial sequence
DILLTQSPVILSVSPGERVSFSCRASQSIGTNIHWYQQRTNGSPRLLIKYASESISGIPSRFSGSGSGTDFTLSINSVESEDIADYYCQQNNNWPTTFGAGTKLELKRTVAAPSVFIFPPSDEQLKSGTASVVCLLNNFYPREAKVQWKVDNALQSGNSQESVTEQDSKDSTYSLSSTLTLSKADYEKHKVYACEVTHQGLSSPVTKSFNRGEC

SEQ ID NO: 58 - protein, 448 aa, Artificial sequence
EVQLVESGGGLVQPGGSLRLSCAASGFTFSDSWIHWVRQAPGKGLEWVAWISPYGGSTYYADSVKGRFTISADTSKNTAYLQMNSLRAEDTAVYYCARRHWPGGFDYWGQGTLVTVSSASTKGPSVFPLAPSSKSTSGGTAALGCLVKDYFPEPVTVSWNSGALTSGVHTFPAVLQSSGLYSLSSVVTVPSSSLGTQTYICNVNHKPSNTKVDKKVEPKSCDKTHTCPPCPAPELLGGPSVFLFPPKPKDTLMISRTPEVTCVVVDVSHEDPEVKFNWYVDGVEVHNAKTKPREEQYASTYRVVSVLTVLAQDWLNGKEYKCKVSNKALPAPIEKTISKAKGQPREPQVYTLPPSREEMTKNQVSLTCLVKGFYPSDIAVEWESNGQPENNYKTTPPVLDSDGSFFLYSKLTVDKSRWQQGNVFSCSVMHEALHNQYTQKSLSLSPGK

SEQ ID NO: 59 - protein, 214 aa, Artificial sequence
DIQMTQSPSSLSASVGDRVTITCRASQDVSTAVAWYQQKPGKAPKLLIYSASFLYSGVPSRFSGSGSGTDFTLTISSLQPEDFATYYCQQYLYHPATFGQGTKVEIKRTVAAPSVFIFPPSDEQLKSGTASVVCLLNNFYPREAKVQWKVDNALQSGNSQESVTEQDSKDSTYSLSSTLTLSKADYEKHKVYACEVTHQGLSSPVTKSFNRGEC

SEQ ID NO: 60 - protein, 450 aa, Artificial sequence
EVQLLESGGGLVQPGGSLRLSCAASGFTFSSYIMMWVRQAPGKGLEWVSSIYPSGGITFYADTVKGRFTISRDNSKNTLYLQMNSLRAEDTAVYYCARIKLGTVTTVDYWGQGTLVTVSSASTKGPSVFPLAPSSKSTSGGTAALGCLVKDYFPEPVTVSWNSGALTSGVHTFPAVLQSSGLYSLSSVVTVPSSSLGTQTYICNVNHKPSNTKVDKKVEPKSCDKTHTCPPCPAPELLGGPSVFLFPPKPKDTLMISRTPEVTCVVVDVSHEDPEVKFNWYVDGVEVHNAKTKPREEQYNSTYRVVSVLTVLHQDWLNGKEYKCKVSNKALPAPIEKTISKAKGQPREPQVYTLPPSRDELTKNQVSLTCLVKGFYPSDIAVEWESNGQPENNYKTTPPVLDSDGSFFLYSKLTVDKSRWQQGNVFSCSVMHEALHNHYTQKSLSLSPGK

SEQ ID NO: 61 - protein, 216 aa, Artificial sequence
QSALTQPASVSGSPGQSITISCTGTSSDVGGYNYVSWYQQHPGKAPKLMIYDVSNRPSGVSNRFSGSKSGNTASLTISGLQAEDEADYYCSSYTSSSTRVFGTGTKVTVLGQPKANPTVTLFPPSSEELQANKATLVCLISDFYPGAVTVAWKADGSPVKAGVETTKPSKQSNNKYAASSYLSLTPEQWKSHRSYSCQVTHEGSTVEKTVAPTECS

SEQ ID NO: 62 - protein, 451 aa, Artificial sequence
EVQLVESGGGLVQPGGSLRLSCAASGFTFSRYWMSWVRQAPGKGLEWVANIKQDGSEKYYVDSVKGRFTISRDNAKNSLYLQMNSLRAEDTAVYYCAREGGWFGELAFDYWGQGTLVTVSSASTKGPSVFPLAPSSKSTSGGTAALGCLVKDYFPEPVTVSWNSGALTSGVHTFPAVLQSSGLYSLSSVVTVPSSSLGTQTYICNVNHKPSNTKVDKRVEPKSCDKTHTCPPCPAPEFEGGPSVFLFPPKPKDTLMISRTPEVTCVVVDVSHEDPEVKFNWYVDGVEVHNAKTKPREEQYNSTYRVVSVLTVLAQDWLNGKEYKCKVSNKALPASIEKTISKAKGQPREPQVYTLPPSREEMTKNQVSLTCLVKGFYPSDIAVEWESNGQPENNYKTTPPVLDSDGSFFLYSKLTVDKSRWQQGNVFSCSVMHEALHNQYTQKSLSLSPGK

SEQ ID NO: 63 - protein, 215 aa, Artificial sequence
EIVLTQSPGTLSLSPGERATLSCRASQRVSSSYLAWYQQKPGQAPRLLIYDASSRATGIPDRFSGSGSGTDFTLTISRLEPEDFAVYYCQQYGSLPWTFGQGTKVEIKRTVAAPSVFIFPPSDEQLKSGTASVVCLLNNFYPREAKVQWKVDNALQSGNSQESVTEQDSKDSTYSLSSTLTLSKADYEKHKVYACEVTHQGLSSPVTKSFNRGEC

SEQ ID NO: 64 - protein, 452 aa, Artificial sequence
EVQLLESGGGLVQPGGSLRLSCAVSGFTFNSFAMSWVRQAPGKGLEWVSAISGSGGGTYYADSVKGRFTISRDNSKNTLYLQMNSLRAEDTAVYFCAKDKILWFGEPVFDYWGQGTLVTVSSASTKGPSVFPLAPSSKSTSGGTAALGCLVKDYFPEPVTVSWNSGALTSGVHTFPAVLQSSGLYSLSSVVTVPSSSLGTQTYICNVNHKPSNTKVDKRVEPKSCDKTHTCPPCPAPELLGGPSVFLFPPKPKDTLMISRTPEVTCVVVDVSHEDPEVKFNWYVDGVEVHNAKTKPREEQYNSTYRVVSVLTVLHQDWLNGKEYKCKVSNKALPAPIEKTISKAKGQPREPQVYTLPPSREEMTKNQVSLTCLVKGFYPSDIAVEWESNGQPENNYKTTPPVLDSDGSFFLYSKLTVDKSRWQQGNVFSCSVMHEALHNHYTQKSLSLSPGK

SEQ ID NO: 65 - protein, 214 aa, Artificial sequence
EIVLTQSPATLSLSPGERATLSCRASQSVSSYLAWYQQKPGQAPRLLIYDASNRATGIPARFSGSGSGTDFTLTISSLEPEDFAVYYCQQRSNWPPTFGQGTKVEIKRTVAAPSVFIFPPSDEQLKSGTASVVCLLNNFYPREAKVQWKVDNALQSGNSQESVTEQDSKDSTYSLSSTLTLSKADYEKHKVYACEVTHQGLSSPVTKSFNRGEC

SEQ ID NO: 66 - protein, 451 aa, Artificial sequence
QVQLVQSGAEVKKPGASVKVSCKGSGYTFTSYWMHWVRQAPGQRLEWIGEIDPSESNTNYNQKFKGRVTLTVDISASTAYMELSSLRSEDTAVYYCARGGYDGWDYAIDYWGQGTLVTVSSASTKGPSVFPLAPSSKSTSGGTAALGCLVKDYFPEPVTVSWNSGALTSGVHTFPAVLQSSGLYSLSSVVTVPSSSLGTQTYICNVNHKPSNTKVDKKVEPKSCDKTHTCPPCPAPELAGAPSVFLFPPKPKDTLMISRTPEVTCVVVDVSHEDPEVKFNWYVDGVEVHNAKTKPREEQYNSTYRVVSVLTVLAQDWLNGKEYKCKVSNKALPAPIEKTISKAKGQPREPQVYTLPPSRDELTKNQVSLTCLVKGFYPSDIAVEWESNGQPENNYKTTPPVLDSDGSFFLYSKLTVDKSRWQQGNVFSCSVMHEALHNQYTQKSLSLSPGK

SEQ ID NO: 67 - protein, 219 aa, Artificial sequence
DVVMTQSPLSLPVTPGEPASISCRSSQSLAKSYGNTYLSWYLQKPGQSPQLLIYGISNRFSGVPDRFSGSGSGTDFTLKISRVEAEDVGVYYCLQGTHQPYTFGQGTKVEIKRTVAAPSVFIFPPSDEQLKSGTASVVCLLNNFYPREAKVQWKVDNALQSGNSQESVTEQDSKDSTYSLSSTLTLSKADYEKHKVYACEVTHQGLSSPVTKSFNRGEC

SEQ ID NO: 68 - protein, 451 aa, Artificial sequence
QVQLQESGPGLVRPSQTLSLTCTVSGFTFTDFYMNWVRQPPGRGLEWIGFIRDKAKGYTTEYNPSVKGRVTMLVDTSKNQFSLRLSSVTAADTAVYYCAREGHTAAPFDYWGQGSLVTVSSASTKGPSVFPLAPSSKSTSGGTAALGCLVKDYFPEPVTVSWNSGALTSGVHTFPAVLQSSGLYSLSSVVTVPSSSLGTQTYICNVNHKPSNTKVDKKVEPKSCDKTHTCPPCPAPELLGGPSVFLFPPKPKDTLMISRTPEVTCVVVDVSHEDPEVKFNWYVDGVEVHNAKTKPREEQYNSTYRVVSVLTVLHQDWLNGKEYKCKVSNKALPAPIEKTISKAKGQPREPQVYTLPPSRDELTKNQVSLTCLVKGFYPSDIAVEWESNGQPENNYKTTPPVLDSDGSFFLYSKLTVDKSRWQQGNVFSCSVMHEALHNHYTQKSLSLSPGK

SEQ ID NO: 69 - protein, 211 aa, Artificial sequence
DIQMTQSPSSLSASVGDRVTITCKASQNIDKYLNWYQQKPGKAPKLLIYNTNNLQTGVPSRFSGSGSGTDFTFTISSLQPEDIATYYCLQHISRPRTFGQGTKVEIKRTVAAPSVFIFPPSDEQLKSGTASVVCLLNNFYPREAKVQWKVDNALQSGNSQESVTEQDSKDSTYSLSSTLTLSKADYEKHKVYACEVTHQGLSSPVTKSFNR

SEQ ID NO: 70 - protein, 449 aa, Artificial sequence
EVQLVESGGDLVQPGRSLRLSCAASGFIFSNYGMSWVRQAPGKGLEWVATISSASTYSYYPDSVKGRFTISRDNAKNSLYLQMNSLRVEDTALYYCGRHSDGNFAFGYWGQGTLVTVSSASTKGPSVFPLAPSSKSTSGGTAALGCLVKDYFPEPVTVSWNSGALTSGVHTFPAVLQSSGLYSLSSVVTVPSSSLGTQTYICNVNHKPSNTKVDKKVEPKSCDKTHTCPPCPAPELLGGPSVFLFPPKPKDTLMISRTPEVTCVVVDVSHEDPEVKFNWYVDGVEVHNAKTKPREEQYNSTYRVVSVLTVLAQDWLNGKEYKCKVSNKALPAPIEKTISKAKGQPREPQVYTLPPSRDELTKNQVSLTCLVKGFYPSDIAVEWESNGQPENNYKTTPPVLDSDGSFFLYSKLTVDKSRWQQGNVFSCSVMHEALHNQYTQKSLSLSPGK

SEQ ID NO: 71 - protein, 229 aa, Artificial sequence
DVLMTQSPLSLPVTPGEPASISCRSSRNIVHINGDTYLEWYLQKPGQSPQLLIYKVSNRFSGVPDRFSGSGSGTDFTLKISRVEAEDVGVYYCFQGSLLPWTFGQGTKVEIKRTVAAPSVFIFPPSDEQLKSGTASVVCLLNNFYPREAKVQWKVDNALQSGNSQESVTEQDSKDSTYSLSSTLTLSKADYEKHKVYACEVTHQGLSSPVTKSFNRGECDACLIZUMAB

SEQ ID NO: 72 - protein, 442 aa, Artificial sequence
QVQLVQSGAEVKKPGSSVKVSCKASGYTFTSYRMHWVRQAPGQGLEWIGYINPSTGYTEYNQKFKDKATITADESTNTAYMELSSLRSEDTAVYYCARGGGVFDYWGQGTTLTVSSGPSVFPLAPSSKSTSGGTAALGCLVKDYFPEPVTVSWNSGALTSGVHTFPAVLQSSGLYSLSSVVTVPSSSLGTQTYICNVNHKPSNTKVDKKAEPKSCDKTHTCPPCPAPELLGGPSVFLFPPKPKDTLMISRTPEVTCVVVDVSHEDPEVKFNWYVDGVEVHNAKTKPREEQYNSTYRVVSVLTVLHQDWLNGKEYKCKVSNKALPAPIEKTISKAKGQPREPQVYTLPPSRDELTKNQVSLTCLVKGFYPSDIAVEWESNGQPENNYKTTPPVLDSDGSFFLYSKLTVDKSRWQQGNVFSCSVMHEALHNHYTQKSLSLSPGK

SEQ ID NO: 73 - protein, 210 aa, Artificial sequence
DIQMTQSPSTLSASVGDRVTITCSASSSISYMHWYQQKPGKAPKLLIYTTSNLASGVPARFSGSGSGTEFTLTISSLQPDDFATYYCHQRSTYPLTFGSGTKVEVKRTVAAPSVFIFPPSDEQLKSGTASVVCLLNNFYPREAKVQWKVDNALQSGNSQESVTEQDSKDSTYSLSSTLTLSKADYEKHKVYACEVTHQGLSSPVTKSFNR

SEQ ID NO: 74 - protein, 446 aa, Artificial sequence
QLQQSGTVLARPGASVKMSCKASGYSFTRYWMHWIKQRPGQGLEWIGAIYPGNSDTSYNQKFEGKAKLTAVTSASTAYMELSSLTHEDSAVYYCSRDYGYYFDFWGQGTTLTVSSASTKGPSVFPLAPSSKSTSGGTAALGCLVKDYFPEPVTVSWNSGALTSGVHTFPAVLQSSGLYSLSSVVTVPSSSLGTQTYICNVNHKPSNTKVDKRVEPPKSCDKTHTCPPCPAPELLGGPSVFLFPPKPKDTLMISRTPEVTCVVVDVSHEDPEVKFNWYVDGVEVHNAKTKPREEQYNSTYRVVSVLTVLAQDWLNGKEYKCKVSNKALPAPIEKTISKAKGQPREPQVYTLPPSRDELTKNQVSLTCLVKGFYPSDIAVEWESNGQPENNYKTTPPVLDSDGSFFLYSKLTVDKSRWQQGNVFSCSVMHEALHNQYTQKSLSLSPGK

SEQ ID NO: 75 - protein, 210 aa, Artificial sequence
QIVSTQSPAIMSASPGEKVTMTCSASSSRSYMQWYQQKPGTSPKRWIYDTSKLASGVPARFSGSGSGTSYSLTISSMEAEDAATYYCHQRSSYTFGGGTKLEIKRTVAAPSVFIFPPSDEQLKSGTASVVCLLNNFYPREAKVQWKVDNALQSGNSQESVTEQDSKDSTYSLSSTLTLSKADYEKHKVYACEVTHQGLSSPVTKSFNRGE

SEQ ID NO: 76 - protein, 443 aa, Artificial sequence
EVQLVQSGAEVKKPGSSVKVSCKASGYTITDSNIHWVRQAPGQSLEWIGYIYPYNGGTDYNQKFKNRATLTVDNPTNTAYMELSSLRSEDTAFYYCVNGNPWLAYWGQGTLVTVSSASTKGPSVFPLAPCSRSTSESTAALGCLVKDYFPEPVTVSWNSGALTSGVHTFPAVLQSSGLYSLSSVVTVPSSSLGTKTYTCNVDHKPSNTKVDKRVESKYGPPCPPCPAPEFLGGPSVFLFPPKPKDTLMISRTPEVTCVVVDVSQEDPEVQFNWYVDGVEVHNAKTKPREEQFNSTYRVVSVLTVLAQDWLNGKEYKCKVSNKGLPSSIEKTISKAKGQPREPQVYTLPPSQEEMTKNQVSLTCLVKGFYPSDIAVEWESNGQPENNYKTTPPVLDSDGSFFLYSRLTVDKSRWQEGNVFSCSVMHEALHNQYTQKSLSLSLGK

SEQ ID NO: 77 - protein, 218 aa, Artificial sequence
DIQLTQSPSTLSASVGDRVTITCRASESLDNYGIRFLTWFQQKPGKAPKLLMYAASNQGSGVPSRFSGSGSGTEFTLTISSLQPDDFATYYCQQTKEVPWSFGQGTKVEVKRTVAAPSVFIFPPSDEQLKSGTASVVCLLNNFYPREAKVQWKVDNALQSGNSQESVTEQDSKDSTYSLSSTLTLSKADYEKHKVYACEVTHQGLSSPVTKSFNRGEC

SEQ ID NO: 78 - protein, 448 aa, Artificial sequence
QVQLVESGGGVVQPGRSLRLSCAASGFTFSSYTMHWVRQAPGKGLEWVTFISYDGNNKYYADSVKGRFTISRDNSKNTLYLQMNSLRAEDTAIYYCARTGWLGPFDYWGQGTLVTVSSASTKGPSVFPLAPSSKSTSGGTAALGCLVKDYFPEPVTVSWNSGALTSGVHTFPAVLQSSGLYSLSSVVTVPSSSLGTQTYICNVNHKPSNTKVDKRVEPKSCDKTHTCPPCPAPELLGGPSVFLFPPKPKDTLMISRTPEVTCVVVDVSHEDPEVKFNWYVDGVEVHNAKTKPREEQYNSTYRVVSVLTVLHQDWLNGKEYKCKVSNKALPAPIEKTISKAKGQPREPQVYTLPPSRDELTKNQVSLTCLVKGFYPSDIAVEWESNGQPENNYKTTPPVLDSDGSFFLYSKLTVDKSRWQQGNVFSCSVMHEALHNHYTQKSLSLSPGK

SEQ ID NO: 79 - protein, 215 aa, Artificial sequence
EIVLTQSPGTLSLSPGERATLSCRASQSVGSSYLAWYQQKPGQAPRLLIYGAFSRATGIPDRFSGSGSGTDFTLTISRLEPEDFAVYYCQQYGSSPWTFGQGTKVEIKRTVAAPSVFIFPPSDEQLKSGTASVVCLLNNFYPREAKVQWKVDNALQSGNSQESVTEQDSKDSTYSLSSTLTLSKADYEKHKVYACEVTHQGLSSPVTKSFNRGEC

SEQ ID NO: 80 - protein, 446 aa, Artificial sequence
EVQLQQSGPELEKPGASVKMSCKASGTSFTGYNMNWVKQSNGKSLEWIGNIDPYYGNTNYNQKFKGKATLTVQKSSSTAYLQLKSLTSEDSAVYYCARLGLQLYAMDYWGQGTSVTVSSASTKGPSVFPLAPCSRSTSESTAALGCLVKDYFPEPVTVSWNSGALTSGVHTFPAVLQSSGLYSLSSVVTVPSSSLGTKTYTCNVDHKPSNTKVDKRVESKYGPPCPSCPAPEFLGGPSVFLFPPKPKDTLMISRTPEVTCVVVDVSQEDPEVQFNWYVDGVEVHNAKTKPREEQFNSTYRVVSVLTVLAQDWLNGKEYKCKVSNKGLPSSIEKTISKAKGQPREPQVYTLPPSQEEMTKNQVSLTCLVKGFYPSDIAVEWESNGQPENNYKTTPPVLDSDGSFFLYSRLTVDKSRWQEGNVFSCSVMHEALHNQYTQKSLSLSLGK

SEQ ID NO: 81 - protein, 112 aa, Artificial sequence
DVVMTQTPLSLPVSLGDQASISCRSSQSLVHSNGNTYLHWYLQKPGQSPNLLIYKLTNRFFGVPDRFSGSGSGTDFTLKISRVEAEDLGVYFCSQSIHVPWTFGGGTKLEIK

SEQ ID NO: 82 - protein, 443 aa, Artificial sequence
QVQLQQSGAELAKPGSSVMISCKASGYTFTNYAVHWIKQTTGQALEWTGYIAPGSGVTKYNEKFKGKATLTYDKSSTTAYMQLSSLTPVDTAVYYCASGTTRFAYWGQGTLVTVSSASTKGPSVFPLAPCSRSTSESTAALGCLVKDYFPEPVTVSWNSGALTSGVHTFPAVLQSSGLYSLSSVVTVPSSSLGTKTYTCNVDHKPSNTKVDKRVESKYGPPCPSCPAPEFLGGPSVFLFPPKPKDTLMISRTPEVTCVVVDVSQEDPEVQFNWYVDGVEVHNAKTKPREEQFNSTYRVVSVLTVLAQDWLNGKEYKCKVSNKGLPSSIEKTISKAKGQPREPQVYTLPPSQEEMTKNQVSLTCLVKGFYPSDIAVEWESNGQPENNYKTTPPVLDSDGSFFLYSRLTVDKSRWQEGNVFSCSVMHEALHNQYTQKSLSLSLGK

SEQ ID NO: 83 - protein, 110 aa, Artificial sequence
DIVLTQSPATAVSLGQRATISCRASQSVSLSSYNLMQINYQQKPGQEPKILIYDASNLPSGIPARFSGSGSGTDFTLTIDPVQADDATYYCQQSKDDPLTFGSGTKLEIK

SEQ ID NO: 84 - protein, 451 aa, Artificial sequence
QVQLVESGGGVVQPGRSLRLSCAASGFTFSSYGMHWVRQAPGKGLEWVAVIWYEGSNKYYADSVKGRFTISRDNSKNTLYLQMNSLRAEDTAVYYCARGGSMVRGDYYYGMDVWGQGTTVTVSSASTKGPSVFPLAPCSRSTSESTAALGCLVKDYFPEPVTVSWNSGALTSGVHTFPAVLQSSGLYSLSSVVTVPSSSLGTKTYTCNVDHKPSNTKVDKRVESKYGPPCPSCPAPEFLGGPSVFLFPPKPKDTLMISRTPEVTCVVVDVSQEDPEVQFNWYVDGVEVHNAKTKPREEQFNSTYRVVSVLTVLAQDWLNGKEYKCKVSNKGLPSSIEKTISKAKGQPREPQVYTLPPSQEEMTKNQVSLTCLVKGFYPSDIAVEWESNGQPENNYKTTPPVLDSDGSFFLYSRLTVDKSRWQEGNVFSCSVMHEALHNQYTQKSLSLSLGK

SEQ ID NO: 85 - protein, 107 aa, Artificial sequence
AIQLTQSPSSLSASVGDRVTITCRASQGISSALAWYQQKPGKAPKLLIYDASSLESGVPSRFSGSGSGTDFTLTISSLQPEDFATYYCQQFNSYPYTFGQGTKLEIK

SEQ ID NO: 86 - protein, 450 aa, Artificial sequence
QVQLVESGGGVVQPGRSLRLSCVASGFTFSSTGMHWVAQRPGKGLEWVAIIWYDGSNKYYADSVKGRFTISRDNSKNTQYLQMNSLRAEDTAVYYCASVATSGDFDYYGMDVWGQGTTVTVSSASTKGPSVFPLAPCSRSTSESTAALGCLVKDYFPEPVTVSWNSGALTSGVHTFPAVLQSSGLYSLSSVVTVPSSSLGTKTYTCNVDHKPSNTKVDKRVESKYGPPCPSCPAPEFLGGPSVFLFPPKPKDTLMISRTPEVTCVVVDVSQEDPEVQFNWYVDGVEVHNAKTKPREEQFNSTYRVVSVLTVLAQDWLNGKEYKCKVSNKGLPSSIEKTISKAKGQPREPQVYTLPPSQEEMTKNQVSLTCLVKGFYPSDIAVEWESNGQPENNYKTTPPVLDSDGSFFLYSRLTVDKSRWQEGNVFSCSVMHEALHNQYTQKSLSLSLGK

SEQ ID NO: 87 - protein, 107 aa, Artificial sequence
EIVLTQSPATLSLSPGERTTLSCRASQRISTTLAWTQQKPGQAPRLLIYDASKRATTGIPARFSGSGSGTGFTLTISSLEEDFAVYYCQQRANWPLTFGGGTKVEIK

SEQ ID NO: 88 - protein, 452 aa, Artificial sequence
QVQLQQSGSELMMPGASVKISCKATGYTFSNYWIEWVKQRPGHGLEWIGEILPGTGRTIYNEKFKGKATFTADISSNTVQMQLSSLTSEDSAVYYCARRDYYGNFYYAMDYWGQGTSVTVSSASTKGPSVFPLAPSSKSTSGGTAALGCLVKDYFPEPVTVSWNSGALTSGVHTFPAVLQSSGLYSLSSVVTVPSSSLGTQTYICNVNHKPSNTKVDKKVEPKSCDKTHTCPPCPAPELLGGPSVFLFPPKPKDTLMISRTPEVTCVVVDVSHEDPEVKFNWYVDGVEVHNAKTKPREEQYNSTYRVVSVLTVLAQDWLNGKEYKCKVSNKALPAPIEKTISKAKGQPREPQVYTLPPSRDELTKNQVSLTCLVKGFYPSDIAVEWESNGQPENNYKTTPPVLDSDGSFFLYSKLTVDKSRWQQGNVFSCSVMHEALHNQYTQKSLSLSPGK

SEQ ID NO: 89 - protein, 214 aa, Artificial sequence
DIQMTQSTSSLSASLGDRVTISCSASQGINNYLNWYQQKPDGTVELLIYYTSTLQSGVPSRFSGSGSGTDYSLTISNLEPEDIGTYYCQQYSKLPRTFGGGTKLEIKRTVAAPSVFIFPPSDEQLKSGTASVVCLLNNFYPREAKVQWKVDNALQSGNSQESVTEQDSKDSTYSLSSTLTLSKADYEKHKVYACEVTHQGLSSPVTKSFNRGEC

SEQ ID NO: 90 - protein, 217 aa, Artificial sequence
APELLGGPSVFLFPPKPKDTLMASRTPEVTCVVVDVSHEDPEVKFNWYVDGVEVHNAKTKPREEQYNSTYRVVSVLTVLHQDWLNGKEYKCKVSNKALPAPIEKTISKAKGQPREPQVYTLPPSRDELTKNQVSLTCLVKGFYPSDIAVEWESNGQPENNYKTTPPVLDSDGSFFLYSKLTVDKSRWQQGNVFSCSVMHEALHNHYTQKSLSLSPGK

SEQ ID NO: 91 - protein, 217 aa, Artificial sequence
APELLGGPSVFLFPPKPKDTLMIARTPEVTCVVVDVSHEDPEVKFNWYVDGVEVHNAKTKPREEQYNSTYRVVSVLTVLHQDWLNGKEYKCKVSNKALPAPIEKTISKAKGQPREPQVYTLPPSRDELTKNQVSLTCLVKGFYPSDIAVEWESNGQPENNYKTTPPVLDSDGSFFLYSKLTVDKSRWQQGNVFSCSVMHEALHNHYTQKSLSLSPGK

SEQ ID NO: 92 - protein, 217 aa, Artificial sequence
APELLGGPSVFLFPPKPKDTLMISATPEVTCVVVDVSHEDPEVKFNWYVDGVEVHNAKTKPREEQYNSTYRVVSVLTVLHQDWLNGKEYKCKVSNKALPAPIEKTISKAKGQPREPQVYTLPPSRDELTKNQVSLTCLVKGFYPSDIAVEWESNGQPENNYKTTPPVLDSDGSFFLYSKLTVDKSRWQQGNVFSCSVMHEALHNHYTQKSLSLSPGK

SEQ ID NO: 93 - protein, 217 aa, Artificial sequence
APELLGGPSVFLFPPKPKDTLMISRTPEVTCVVVDVSHEDPEVKFNWYVDGVEVHNAATKPREEQYNSTYRVVSVLTVLHQDWLNGKEYKCKVSNKALPAPIEKTISKAKGQPREPQVYTLPPSRDELTKNQVSLTCLVKGFYPSDIAVEWESNGQPENNYKTTPPVLDSDGSFFLYSKLTVDKSRWQQGNVFSCSVMHEALHNHYTQKSLSLSPGK

SEQ ID NO: 94 - protein, 217 aa, Artificial sequence
APELLGGPSVFLFPPKPKDTLMISRTPEVTCVVVDVSHEDPEVKFNWYVDGVEVHNAKTKPREEQYNSTYRVVSVLTVAHQDWLNGKEYKCKVSNKALPAPIEKTISKAKGQPREPQVYTLPPSRDELTKNQVSLTCLVKGFYPSDIAVEWESNGQPENNYKTTPPVLDSDGSFFLYSKLTVDKSRWQQGNVFSCSVMHEALHNHYTQKSLSLSPGK

SEQ ID NO: 95 - protein, 217 aa, Artificial sequence
APELLGGPSVFLFPPKPKDTLMISRTPEVTCVVVDVSHEDPEVKFNWYVDGVEVHNAKTKPREEQYNSTYRVVSVLTVLAQDWLNGKEYKCKVSNKALPAPIEKTISKAKGQPREPQVYTLPPSRDELTKNQVSLTCLVKGFYPSDIAVEWESNGQPENNYKTTPPVLDSDGSFFLYSKLTVDKSRWQQGNVFSCSVMHEALHNHYTQKSLSLSPGK

SEQ ID NO: 96 - protein, 217 aa, Artificial sequence
APELLGGPSVFLFPPKPKDTLMISRTPEVTCVVVDVSHEDPEVKFNWYVDGVEVHNAKTKPREEQYNSTYRVVSVLTVLHQDWLNGKEYKCKVSNKALPAPIEKTISKAKGQPREPQVYTLPPSRDELTKNQVSLTCLVKGFYPSDIAVEWESNGQPENNYKTTPPVLDSDGSFFLYSKLTVDKARWQQGNVFSCSVMHEALHNHYTQKSLSLSPGK

SEQ ID NO: 97 - protein, 217 aa, Artificial sequence
APELLGGPSVFLFPPKPKDTLMISRTPEVTCVVVDVSHEDPEVKFNWYVDGVEVHNAKTKPREEQYNSTYRVVSVLTVLHQDWLNGKEYKCKVSNKALPAPIEKTISKAKGQPREPQVYTLPPSRDELTKNQVSLTCLVKGFYPSDIAVEWESNGQPENNYKTTPPVLDSDGSFFLYSKLTVDKSRWQQGNVFSCSVMHEALANHYTQKSLSLSPGK

SEQ ID NO: 98 - protein, 217 aa, Artificial sequence
APELLGGPSVFLFPPKPKDTLMISRTPEVTCVVVDVSHEDPEVKFNWYVDGVEVHNAKTKPREEQYNSTYRVVSVLTVLHQDWLNGKEYKCKVSNKALPAPIEKTISKAKGQPREPQVYTLPPSRDELTKNQVSLTCLVKGFYPSDIAVEWESNGQPENNYKTTPPVLDSDGSFFLYSKLTVDKSRWQQGNVFSCSVMHEALHNAYTQKSLSLSPGK

SEQ ID NO: 99 - protein, 217 aa, Artificial sequence
APELLGGPSVFLFPPKPKDTLMISRTPEVTCVVVDVSHEDPEVKFNWYVDGVEVHNAKTKPREEQYNSTYRVVSVLTVLHQDWLNGKEYKCKVSNKALPAPIEKTISKAKGQPREPQVYTLPPSRDELTKNQVSLTCLVKGFYPSDIAVEWESNGQPENNYKTTPPVLDSDGSFFLYSKLTVDKSRWQQGNVFSCSVMHEALHNRYTQKSLSLSPGK

SEQ ID NO: 100 - protein, 217 aa, Artificial sequence
APELLGGPSVFLFPPKPKDTLMISRTPEVTCVVVDVSHEDPEVKFNWYVDGVEVHNAKTKPREEQYNSTYRVVSVLTVLHQDWLNGKEYKCKVSNKALPAPIEKTISKAKGQPREPQVYTLPPSRDELTKNQVSLTCLVKGFYPSDIAVEWESNGQPENNYKTTPPVLDSDGSFFLYSKLTVDKSRWQQGNVFSCSVMHEALHNHATQKSLSLSPGK

SEQ ID NO: 101 - protein, 217 aa, Artificial sequence
APELLGGPSVFLFPPKPKDTLMISRTPEVTCVVVDVSHEDPEVKFNWYVDGVEVHNAKTKPREEQYNSTYRVVSVLTVLQQDWLNGKEYKCKVSNKALPAPIEKTISKAKGQPREPQVYTLPPSRDELTKNQVSLTCLVKGFYPSDIAVEWESNGQPENNYKTTPPVLDSDGSFFLYSKLTVDKSRWQQGNVFSCSVMHEALNNHYTQKSLSLSPGK

SEQ ID NO: 102 - protein, 217 aa, Artificial sequence
APELLGGPSVFLFPPKPKDTLYISRQPEVTCVVVDVSHEDPEVKFNWYVDGVEVHNAKTKPREEQYNSTYRVVSVLTVLHQDWLNGKEYKCKVSNKALPAPIEKTISKAKGQPREPQVYTLPPSRDELTKNQVSLTCLVKGFYPSDIAVEWESNGQPENNYKTTPPVLDSDGSFFLYSKLTVDKSRWQQGNVFSCSVMHEALHNHYTQKSLSLSPGK

SEQ ID NO: 103 - protein, 217 aa, Artificial sequence
APELLGGPSVFLFPPKPKDTLFISRDPEVTCVVVDVSHEDPEVKFNWYVDGVEVHNAKTKPREEQYNSTYRVVSVLTVLHQDWLNGKEYKCKVSNKALPAPIEKTISKAKGQPREPQVYTLPPSRDELTKNQVSLTCLVKGFYPSDIAVEWESNGQPENNYKTTPPVLDSDGSFFLYSKLTVDKSRWQQGNVFSCSVMHEALHNHYTQKSLSLSPGK

SEQ ID NO: 104 - protein, 216 aa, Artificial sequence
APPVAGPSVFLFPPKPKDTLMASRTPEVTCVVVDVSHEDPEVQFNWYVDGVEVHNAKTKPREEQFNSTFRVVSVLTVVHQDWLNGKEYKCKVSNKGLPAPIEKTISKTKGQPREPQVYTLPPSREEMTKNQVSLTCLVKGFYPSDISVEWESNGQPENNYKTTPPMLDSDGSFFLYSKLTVDKSRWQQGNVFSCSVMHEALHNHYTQKSLSLSPGK

SEQ ID NO: 105 - protein, 216 aa, Artificial sequence
APPVAGPSVFLFPPKPKDTLMIARTPEVTCVVVDVSHEDPEVQFNWYVDGVEVHNAKTKPREEQFNSTFRVVSVLTVVHQDWLNGKEYKCKVSNKGLPAPIEKTISKTKGQPREPQVYTLPPSREEMTKNQVSLTCLVKGFYPSDISVEWESNGQPENNYKTTPPMLDSDGSFFLYSKLTVDKSRWQQGNVFSCSVMHEALHNHYTQKSLSLSPGK

SEQ ID NO: 106 - protein, 216 aa, Artificial sequence
APPVAGPSVFLFPPKPKDTLMISATPEVTCVVVDVSHEDPEVQFNWYVDGVEVHNAKTKPREEQFNSTFRVVSVLTVVHQDWLNGKEYKCKVSNKGLPAPIEKTISKTKGQPREPQVYTLPPSREEMTKNQVSLTCLVKGFYPSDISVEWESNGQPENNYKTTPPMLDSDGSFFLYSKLTVDKSRWQQGNVFSCSVMHEALHNHYTQKSLSLSPGK

SEQ ID NO: 107 - protein, 216 aa, Artificial sequence
APPVAGPSVFLFPPKPKDTLMISRTPEVTCVVVDVSHEDPEVQFNWYVDGVEVHNAATKPREEQFNSTFRVVSVLTVVHQDWLNGKEYKCKVSNKGLPAPIEKTISKTKGQPREPQVYTLPPSREEMTKNQVSLTCLVKGFYPSDISVEWESNGQPENNYKTTPPMLDSDGSFFLYSKLTVDKSRWQQGNVFSCSVMHEALHNHYTQKSLSLSPGK

SEQ ID NO: 108 - protein, 216 aa, Artificial sequence
APPVAGPSVFLFPPKPKDTLMISRTPEVTCVVVDVSHEDPEVQFNWYVDGVEVHNAKTKPREEQFNSTFRVVSVLTVVAQDWLNGKEYKCKVSNKGLPAPIEKTISKTKGQPREPQVYTLPPSREEMTKNQVSLTCLVKGFYPSDISVEWESNGQPENNYKTTPPMLDSDGSFFLYSKLTVDKSRWQQGNVFSCSVMHEALHNHYTQKSLSLSPGK

SEQ ID NO: 109 - protein, 216 aa, Artificial sequence
APPVAGPSVFLFPPKPKDTLMISRTPEVTCVVVDVSHEDPEVQFNWYVDGVEVHNAKTKPREEQFNSTFRVVSVLTVVHQDWLNGKEYKCKVSNKGLPAPIEKTISKTKGQPREPQVYTLPPSREEMTKNQVSLTCLVKGFYPSDISVEWESNGQPENNYKTTPPMLDSDGSFFLYSKLTVDKARWQQGNVFSCSVMHEALHNHYTQKSLSLSPGK

SEQ ID NO: 110 - protein, 216 aa, Artificial sequence
APPVAGPSVFLFPPKPKDTLMISRTPEVTCVVVDVSHEDPEVQFNWYVDGVEVHNAKTKPREEQFNSTFRVVSVLTVVHQDWLNGKEYKCKVSNKGLPAPIEKTISKTKGQPREPQVYTLPPSREEMTKNQVSLTCLVKGFYPSDISVEWESNGQPENNYKTTPPMLDSDGSFFLYSKLTVDKSRWQQGNVFSCSVMHEALANHYTQKSLSLSPGK

SEQ ID NO: 111 - protein, 216 aa, Artificial sequence
APPVAGPSVFLFPPKPKDTLMISRTPEVTCVVVDVSHEDPEVQFNWYVDGVEVHNAKTKPREEQFNSTFRVVSVLTVVHQDWLNGKEYKCKVSNKGLPAPIEKTISKTKGQPREPQVYTLPPSREEMTKNQVSLTCLVKGFYPSDISVEWESNGQPENNYKTTPPMLDSDGSFFLYSKLTVDKSRWQQGNVFSCSVMHEALHNAYTQKSLSLSPGK

SEQ ID NO: 112 - protein, 216 aa, Artificial sequence
APPVAGPSVFLFPPKPKDTLMISRTPEVTCVVVDVSHEDPEVQFNWYVDGVEVHNAKTKPREEQFNSTFRVVSVLTVVHQDWLNGKEYKCKVSNKGLPAPIEKTISKTKGQPREPQVYTLPPSREEMTKNQVSLTCLVKGFYPSDISVEWESNGQPENNYKTTPPMLDSDGSFFLYSKLTVDKSRWQQGNVFSCSVMHEALHNRYTQKSLSLSPGK

SEQ ID NO: 113 - protein, 216 aa, Artificial sequence
APPVAGPSVFLFPPKPKDTLMISRTPEVTCVVVDVSHEDPEVQFNWYVDGVEVHNAKTKPREEQFNSTFRVVSVLTVVHQDWLNGKEYKCKVSNKGLPAPIEKTISKTKGQPREPQVYTLPPSREEMTKNQVSLTCLVKGFYPSDISVEWESNGQPENNYKTTPPMLDSDGSFFLYSKLTVDKSRWQQGNVFSCSVMHEALHNHATQKSLSLSPGK

SEQ ID NO: 114 - protein, 216 aa, Artificial sequence
APPVAGPSVFLFPPKPKDTLMISRTPEVTCVVVDVSHEDPEVQFNWYVDGVEVHNAKTKPREEQFNSTFRVVSVLTVVQQDWLNGKEYKCKVSNKGLPAPIEKTISKTKGQPREPQVYTLPPSREEMTKNQVSLTCLVKGFYPSDISVEWESNGQPENNYKTTPPMLDSDGSFFLYSKLTVDKSRWQQGNVFSCSVMHEALHNNYTQKSLSLSPGK

SEQ ID NO: 115 - protein, 216 aa, Artificial sequence
APPVAGPSVFLFPPKPKDTLYISRQPEVTCVVVDVSHEDPEVQFNWYVDGVEVHNAKTKPREEQFNSTFRVVSVLTVVHQDWLNGKEYKCKVSNKGLPAPIEKTISKTKGQPREPQVYTLPPSREEMTKNQVSLTCLVKGFYPSDISVEWESNGQPENNYKTTPPMLDSDGSFFLYSKLTVDKSRWQQGNVFSCSVMHEALHNHYTQKSLSLSPGK

SEQ ID NO: 116 - protein, 216 aa, Artificial sequence
APPVAGPSVFLFPPKPKDTLFISRDPEVTCVVVDVSHEDPEVQFNWYVDGVEVHNAKTKPREEQFNSTFRVVSVLTVVHQDWLNGKEYKCKVSNKGLPAPIEKTISKTKGQPREPQVYTLPPSREEMTKNQVSLTCLVKGFYPSDISVEWESNGQPENNYKTTPPMLDSDGSFFLYSKLTVDKSRWQQGNVFSCSVMHEALHNHYTQKSLSLSPGK

SEQ ID NO: 117 - protein, 217 aa, Artificial sequence
APEFLGGPSVFLFPPKPKDTLMASRTPEVTCVVVDVSQEDPEVQFNWYVDGVEVHNAKTKPREEQFNSTYRVVSVLTVLHQDWLNGKEYKCKVSNKGLPSSIEKTISKAKGQPREPQVYTLPPSQEEMTKNQVSLTCLVKGFYPSDIAVEWESNGQPENNYKTTPPVLDSDGSFFLYSRLTVDKSRWQEGNVFSCSVMHEALHNHYTQKSLSLSLGK

SEQ ID NO: 118 - protein, 217 aa, Artificial sequence
APEFLGGPSVFLFPPKPKDTLMIARTPEVTCVVVDVSQEDPEVQFNWYVDGVEVHNAKTKPREEQFNSTYRVVSVLTVLHQDWLNGKEYKCKVSNKGLPSSIEKTISKAKGQPREPQVYTLPPSQEEMTKNQVSLTCLVKGFYPSDIAVEWESNGQPENNYKTTPPVLDSDGSFFLYSRLTVDKSRWQEGNVFSCSVMHEALHNHYTQKSLSLSLGK

SEQ ID NO: 119 - protein, 217 aa, Artificial sequence
APEFLGGPSVFLFPPKPKDTLMISATPEVTCVVVDVSQEDPEVQFNWYVDGVEVHNAKTKPREEQFNSTYRVVSVLTVLHQDWLNGKEYKCKVSNKGLPSSIEKTISKAKGQPREPQVYTLPPSQEEMTKNQVSLTCLVKGFYPSDIAVEWESNGQPENNYKTTPPVLDSDGSFFLYSRLTVDKSRWQEGNVFSCSVMHEALHNHYTQKSLSLSLGK

SEQ ID NO: 120 - protein, 217 aa, Artificial sequence
APEFLGGPSVFLFPPKPKDTLMISRTPEVTCVVVDVSQEDPEVQFNWYVDGVEVHNAATKPREEQFNSTYRVVSVLTVLHQDWLNGKEYKCKVSNKGLPSSIEKTISKAKGQPREPQVYTLPPSQEEMTKNQVSLTCLVKGFYPSDIAVEWESNGQPENNYKTTPPVLDSDGSFFLYSRLTVDKSRWQEGNVFSCSVMHEALHNHYTQKSLSLSLGK

SEQ ID NO: 121 - protein, 217 aa, Artificial sequence
APEFLGGPSVFLFPPKPKDTLMISRTPEVTCVVVDVSQEDPEVQFNWYVDGVEVHNAKTKPREEQFNSTYRVVSVLTVAHQDWLNGKEYKCKVSNKGLPSSIEKTISKAKGQPREPQVYTLPPSQEEMTKNQVSLTCLVKGFYPSDIAVEWESNGQPENNYKTTPPVLDSDGSFFLYSRLTVDKSRWQEGNVFSCSVMHEALHNHYTQKSLSLSLGK

SEQ ID NO: 122 - protein, 217 aa, Artificial sequence
APEFLGGPSVFLFPPKPKDTLMISRTPEVTCVVVDVSQEDPEVQFNWYVDGVEVHNAKTKPREEQFNSTYRVVSVLTVLAQDWLNGKEYKCKVSNKGLPSSIEKTISKAKGQPREPQVYTLPPSQEEMTKNQVSLTCLVKGFYPSDIAVEWESNGQPENNYKTTPPVLDSDGSFFLYSRLTVDKSRWQEGNVFSCSVMHEALHNHYTQKSLSLSLGK

SEQ ID NO: 123 - protein, 217 aa, Artificial sequence
APEFLGGPSVFLFPPKPKDTLMISRTPEVTCVVVDVSQEDPEVQFNWYVDGVEVHNAKTKPREEQFNSTYRVVSVLTVLHQDWLNGKEYKCKVSNKGLPSSIEKTISKAKGQPREPQVYTLPPSQEEMTKNQVSLTCLVKGFYPSDIAVEWESNGQPENNYKTTPPVLDSDGSFFLYSRLTVDKARWQEGNVFSCSVMHEALHNHYTQKSLSLSLGK

SEQ ID NO: 124 - protein, 217 aa, Artificial sequence
APEFLGGPSVFLFPPKPKDTLMISRTPEVTCVVVDVSQEDPEVQFNWYVDGVEVHNAKTKPREEQFNSTYRVVSVLTVLHQDWLNGKEYKCKVSNKGLPSSIEKTISKAKGQPREPQVYTLPPSQEEMTKNQVSLTCLVKGFYPSDIAVEWESNGQPENNYKTTPPVLDSDGSFFLYSRLTVDKSRWQEGNVFSCSVMHEALANHYTQKSLSLSLGK

SEQ ID NO: 125 - protein, 217 aa, Artificial sequence
APEFLGGPSVFLFPPKPKDTLMISRTPEVTCVVVDVSQEDPEVQFNWYVDGVEVHNAKTKPREEQFNSTYRVVSVLTVLHQDWLNGKEYKCKVSNKGLPSSIEKTISKAKGQPREPQVYTLPPSQEEMTKNQVSLTCLVKGFYPSDIAVEWESNGQPENNYKTTPPVLDSDGSFFLYSRLTVDKSRWQEGNVFSCSVMHEALHNAYTQKSLSLSLGK

SEQ ID NO: 126 - protein, 217 aa, Artificial sequence
APEFLGGPSVFLFPPKPKDTLMISRTPEVTCVVVDVSQEDPEVQFNWYVDGVEVHNAKTKPREEQFNSTYRVVSVLTVLHQDWLNGKEYKCKVSNKGLPSSIEKTISKAKGQPREPQVYTLPPSQEEMTKNQVSLTCLVKGFYPSDIAVEWESNGQPENNYKTTPPVLDSDGSFFLYSRLTVDKSRWQEGNVFSCSVMHEALHNRYTQKSLSLSLGK

SEQ ID NO: 127 - protein, 217 aa, Artificial sequence
APEFLGGPSVFLFPPKPKDTLMISRTPEVTCVVVDVSQEDPEVQFNWYVDGVEVHNAKTKPREEQFNSTYRVVSVLTVLHQDWLNGKEYKCKVSNKGLPSSIEKTISKAKGQPREPQVYTLPPSQEEMTKNQVSLTCLVKGFYPSDIAVEWESNGQPENNYKTTPPVLDSDGSFFLYSRLTVDKSRWQEGNVFSCSVMHEALHNHATQKSLSLSLGK

SEQ ID NO: 128 - protein, 217 aa, Artificial sequence
APEFLGGPSVFLFPPKPKDTLMISRTPEVTCVVVDVSQEDPEVQFNWYVDGVEVHNAKTKPREEQFNSTYRVVSVLTVLQQDWLNGKEYKCKVSNKGLPSSIEKTISKAKGQPREPQVYTLPPSQEEMTKNQVSLTCLVKGFYPSDIAVEWESNGQPENNYKTTPPVLDSDGSFFLYSRLTVDKSRWQEGNVFSCSVMHEALHNNYTQKSLSLSLGK

SEQ ID NO: 129 - protein, 217 aa, Artificial sequence
APEFLGGPSVFLFPPKPKDTLYISRQPEVTCVVVDVSQEDPEVQFNWYVDGVEVHNAKTKPREEQFNSTYRVVSVLTVLHQDWLNGKEYKCKVSNKGLPSSIEKTISKAKGQPREPQVYTLPPSQEEMTKNQVSLTCLVKGFYPSDIAVEWESNGQPENNYKTTPPVLDSDGSFFLYSRLTVDKSRWQEGNVFSCSVMHEALHNHYTQKSLSLSLGK

SEQ ID NO: 130 - protein, 217 aa, Artificial sequence
APEFLGGPSVFLFPPKPKDTLFISRDPEVTCVVVDVSQEDPEVQFNWYVDGVEVHNAKTKPREEQFNSTYRVVSVLTVLHQDWLNGKEYKCKVSNKGLPSSIEKTISKAKGQPREPQVYTLPPSQEEMTKNQVSLTCLVKGFYPSDIAVEWESNGQPENNYKTTPPVLDSDGSFFLYSRLTVDKSRWQEGNVFSCSVMHEALHNHYTQKSLSLSLGK

SEQ ID NO: 131 - protein, 197 aa, Artificial sequence
ANLPVATPDPGMFPCLHHSQNLLRAVSNMLQKARQTLEFYPCTSEEIDHEDITKDKTSTVEACLPLELTKNESCLNSRETSFITNGSCLASRKTSFMMALCLSSIYEDLKMYQVEFKTMNAKLLMDPKRQIFLDQNMLAVIDELMQALNFNSETVPQKSSLEEPDFYKTKIKLCILLHAFRIRAVTIDRVMSYLNAS

SEQ ID NO: 132 - protein, 327 aa, Artificial sequence
MCHQQLVISWFSLVFLASPLVAIWELKKDVYVVELDWYPDAPGEMVVLTCDTPEEDGITWTLDQSSEVLGSGKTLTIQVKEFGDAGQYTCHKGGEVLSHSLLLLHKKEDGIWSTDILKDQKEPKNKTFLRCEAKNYSGRFTCWWLTTISTDLTFSVKSSRGSSDPQGVTCGAATLSAERVRGDNKEYEYSVECQEDSACPAAEESLPIEVMVDAVHKLKYENYTSSFFIRDIIKPDPPKNLQLKPLKNSRQVEVSWEYPDTWSTPHSYFSLTFCVQVQGKDNTEGGRVFTDKTSATVICRKNASISVRAQDRYYSSSWSEWASVPCS

SEQ ID NO: 133 - protein, 100 aa, Artificial sequence
PKKKIQLHAEHALYDALMILNIVKTNSPPAEEKLEDYAFNFELILEEIARLFESGDQKDEAEKAKRMKEWMKRIKTTASEDEQEEMANAIITILQSWIFS

SEQ ID NO: 134 - protein, 152 aa, Artificial sequence
DCDIEGKDGKQYESVLMVSIDQLLDSMKEIGSNCLNNEFNFFKRHICDANKEGMFLFRAARKLRQFLKMNSTGDFDLHLLKVSEGTTILLNCTGQVKGRKPAALGEAQPTKSLEENKSLKEQKKLNDLCFLKRLLQEIKTCWNKILMGTKEH

SEQ ID NO: 135 - protein, 157 aa, Artificial sequence
YFGKLESKLSVIRNLNDQVLFIDQGNRPLFEDMTDSDCRDNAPRTIFIISMYKDSQPRGMAVTISVKCEKISTLSCENKIISFKEMNPPDNIKDTKSDIIFFQRSVPGHDNKMQFESSSYEGYFLACEKERDLFKLILKKEDELGDRSIMFTVQNED

SEQ ID NO: 136 - protein, 138 aa, Artificial sequence
HKSSSQGQDRHMIRMRQLIDIVDQLKNYVNDLVPEFLPAPEDVETNCEWSAFSCFQKAQLKSANTGNNERIINVSIKKLKRKPPSTNAGRRQKHRLTCPSCDSYEKKPPKEFLERFKSLLQKMIHQHLSSRTHGSEDS

SEQ ID NO: 137 - protein, 364 aa, Artificial sequence
APTSSSTKKTQLQLEHLLLDLQMILNGINNYKNPKLTRMLTFKFYMPKKATELKHLQCLEEELKPLEEVLNLAQSKNFHLRPRDLISNINVIVLELKGSETTFMCEYADETATIVEFLNRWITFAQSIISTLTGGGSGGGSGGGSELCDDDPPEIPHATFKAMAYKEGTMLNCECKRGFRRIKSGSLYMLCTGNSSHSSWDNQCQCTSSATRNTTKQVTPQPEEQKERKTTEMQSPMQPVDQASLPGHCREPPPWENEATERIYHFVVGQMVYYQCVQGYRALHRGPAESVCKMTHGKTRWTQPQLICTGEMETSQFPGEEKPQASPEGRPESETSSLVTTTDFQIQTEMAATMETSIFTTEYQ

SEQ ID NO: 138 - protein, 311 aa, Artificial sequence
APTSSSTKKTQLQLEHLLLDLQMILNGINNYKNPKLTRMLTFKFYMPKKATELKHLQCLEEELKPLEEVLNLAQSKNFHLRPRDLISNINVIVLELKGSETTFMCEYADETATIVEFLNRWITFCQSIISTLTGGGSGGGSGGGSELCDDDPPEIPHATFKAMAYKEGTMLNCECKRGFRRIKSGSLYMLCTGNSSHSSWDNQCQCTSSATRNTTKQVTPQPEEQKERKTTEMQSPMQPVDQASLPGHCREPPPWENEATERIYHFVVGQMVYYQCVQGYRALHRGPAESVCKMTHGKTRWTQPQLICTGE

SEQ ID NO: 139 - protein, 335 aa, Artificial sequence
APTSSSTKKTQLQLEHLLLDLQMILNGINNYKNPKLTRMLTFKFYMPKKATELKHLQCLEEELKPLEEVLNLAQSKNFHLRPRDLISNINVIVLELKGSETTFMCEYADETATIVEFLNRWITFCQSIISTLTGGGSGGGSGGGSELCDDDPPEIPHATFKAMAYKEGTMLNCECKRGFRRIKSGSLYMLCTGNSSHSSWDNQCQCTSSATRNTTKQVTPQPEEQKERKTTEMQSPMQPVDQASLPGHCREPPPWENEATERIYHFWGQMVYYQCVQGYRALHRGPAESVCKMTHGKTRWTQPQLICTGEMETSQFPGEEKPQASPEGRPESETS

SEQ ID NO: 140 - protein, 166 aa, Artificial sequence
CDLPETHSLDNRRTLMLLAQMSRISPSSCLMDRHDFGFPQEEFDGNQFQKAPAISVLHELIQQIFNLFTTKDSSAAWDEDLLDKFCTELYQQLNDLEACVMQEERVGETPLMNADSILAVKKYFRRITLYLTEKKYSPCAWEVVRAEIMRSLSLSTNLQERLRRKE

SEQ ID NO: 141 - protein, 165 aa, Artificial sequence [sequence omitted]

SEQ ID NO: 142 - protein, 165 aa, Artificial sequence
CDLPQTHSLGSRRTLMLLAQMRRQSLFSCLKDRHDFGFPQEEFGNQFQKAETIPVLHEMTQQIANLFSTKDSSAAHDETLLDKFYTELYQQLNDLEACVIQGVGVTETPLMKEDSRLAVRKYFQRITNYLKEKKYSPCAWEVVRAEIMRSFSLSTNLQESLRSKE

SEQ ID NO: 143 - protein, 138 aa, Artificial sequence
QDPYVKEAENLKKYFNAGHSDVADNGTLFLGILKNWKEESDRKIMQSQIVSFYFKLFKNFKDDQSIQKSVETIKEDMNVKFFNSNKKKRDDFEKLTNYSVTDLNVQRKAIHELIQVMAELSPAAKTGKRKRSQMLFRG

SEQ ID NO: 144 - protein, 157 aa, Artificial sequence [sequence omitted]

SEQ ID NO: 145 - protein, 127 aa, Artificial sequence [sequence omitted]

SEQ ID NO: 146 - protein, 209 aa, Artificial sequence
TQDCSFQHSPISSDFAVKIRELSDYLLQDYPVTVASNLQDEELCGGLWRLVLAQRWMERLKTVAGSKMQGLLERVNTEIHFVTKCAFQPPPSCLRFVQTNISRLLQETSEQLVALKPWITRQNFSRCLELQCQPDSSTLPPPWSPRPLEATAPTAPQPPLLLLLLLPVGLLLLAAAWCLHWQRTRRRTPRPGEQVPPVPSPQDLLLVEH

SEQ ID NO: 147 - protein, 111 aa, Artificial sequence
SDGGAQDCCLKYSQRKIPAKVVRSYRKQEPSLGCSIPAILFLPRKRSQAELCADPKELWVQQLMQHLDKTPSPQKPAQGCRKDRGASKTGKKGKGSKGCKRTERSQTPKGP